European Patent Specification EP 3 490 373 B1, published October 25, 2023. Title: FIBRILLIN-1 MUTATIONS FOR MODELING NEONATAL PROGEROID SYNDROME WITH CONGENITAL LIPODYSTROPHY. Applicant: Regeneron Pharmaceuticals, Inc. The sequence listing filed with the application follows.

SEQUENCE LISTING (47 sequences)

SEQ ID NO: 1 - DNA, 24 bp, Homo sapiens
cggagaagcacaaacgaaactgat

SEQ ID NO: 2 - protein, 8 aa, Homo sapiens
RRSTNETD

SEQ ID NO: 3 - DNA, 24 bp, Homo sapiens
cggagaagcacaaacgaaaactga

SEQ ID NO: 4 - protein, 7 aa, Homo sapiens
RRSTNEN

SEQ ID NO: 5 - DNA, 24 bp, Mus musculus
cggagaagcacgaacgaaacggat

SEQ ID NO: 6 - protein, 8 aa, Mus musculus
RRSTNETD

SEQ ID NO: 7 - DNA, 24 bp, Artificial Sequence
  Synthetic
cggagaagcacgaacgaaaactga

SEQ ID NO: 8 - protein, 7 aa, Artificial Sequence
  Synthetic
RRSTNEN

SEQ ID NO: 9 - DNA, 60 bp, Homo sapiens
gagtgtaagatcaatggctaccccaaacggggcaggaaacggagaagcacaaacgaaact

SEQ ID NO: 10 - protein, 20 aa, Homo sapiens
ECKINGYPKRGRKRRSTNET

SEQ ID NO: 11 - DNA, 60 bp, Homo sapiens
gagtgtgatcaatggctaccccaaacggggcaggaaacggagaagcacaaacgaaactga

SEQ ID NO: 12 - protein, 19 aa, Homo sapiens
ECDQWLPQTGQETEKHKRN

SEQ ID NO: 13 - DNA, 60 bp, Mus musculus
gagtgtaagatcaacggctacccaaaacgaggccggaaacggagaagcacgaacgaaacg

SEQ ID NO: 14 - protein, 20 aa, Mus musculus
ECKINGYPKRGRKRRSTNET

SEQ ID NO: 15 - DNA, 60 bp, Artificial Sequence; identical to SEQ ID NO: 11
  Synthetic

SEQ ID NO: 16 - protein, 19 aa, Artificial Sequence
  Synthetic
ECDQWLPQTGQETEKHKRN

SEQ ID NO: 17 - protein, 55 aa, Artificial Sequence
  Synthetic
PPASSEMDDNSLSPEACYECKINGYPKAAQSHLPATRPETEKHERNGCLRHPGRV

SEQ ID NO: 18 - protein, 37 aa, Artificial Sequence
  Synthetic
PPASSEMDDNSLSPEACYECDQWLPQTGQETEKHKRN

SEQ ID NO: 19 - DNA, 8616 bp, Homo sapiens
atgcgtcgagggcgtctgctggagatcgccctgggatttaccgtgcttttagcgtcctacacgagccatggggcggacgccaatttggaggctgggaacgtgaaggaaaccagagccagtcgggccaagagaagaggcggtggaggacacgacgcgcttaaaggacccaatgtctgtggatcacgttataatgcttactgttgccctggatggaaaaccttacctggcggaaatcagtgtattgtccccatttgccggcattcctgtggggatggattttgttcgaggccaaatatgtgcacttgcccatctggtcagatagctccttcctgtggctccagatccatacaacactgcaatattcgctgtatgaatggaggtagctgcagtgacgatcactgtctatgccagaaaggatacatagggactcactgtggacaacctgtttgtgaaagtggctgtctcaatggaggaaggtgtgtggccccaaatcgatgtgcatgcacttacggatttactggaccccagtgtgaaagagattacaggacaggcccatgttttactgtgatcagcaaccagatgtgccagggacaactcagcgggattgtctgcacaaaaacgctctgctgtgccacagtcggccgagcctggggccacccctgtgagatgtgtcctgcccagcctcacccctgccgccgtggcttcattccaaatatccgcacgggagcttgtcaagatgtggatgaatgccaggccatccccgggctctgtcagggaggaaattgcattaatactgttgggtcttttgagtgcaaatgccctgctggacacaaacttaatgaagtgtcacaaaaatgtgaagatattgatgaatgcagcaccattcctggaatctgtgaagggggtgaatgtacaaacacagtcagcagttacttttgcaaatgtccccctggtttttacacctctccagatggtaccagatgcatagatgttcgcccaggatactgttacacagctctgacaaacgggcgctgctctaaccagctgccacagtccataaccaaaatgcagtgctgctgtgatgccggccgatgctggtctccaggggtcactgtcgcccctgagatgtgtcccatcagagcaaccgaggatttcaacaagctgtgctctgttcctatggtaattcctgggagaccagaatatcctcccccaccccttggccccattcctccagttctccctgttcctcctggctttcctcctggacctcaaattccggtccctcgaccaccagtggaatatctgtatccatctcgggagccaccaagggtgctgccagtaaacgttactgattactgccagttggtccgctatctctgtcaaaatggacgctgcattccaactcctgggagttaccggtgtgagtgcaacaaagggttccagctggacctccgtggggagtgtattgatgttgatgaatgtgagaaaaacccctgtgctggtggtgagtgtattaacaaccagggttcgtacacctgtcagtgccgagctggatatcagagcacactcacgcggacagaatgccgagacattgatgagtgtttacagaatggccggatctgcaataatggacgctgcatcaacacagatggcagttttcattgcgtgtgtaatgcgggctttcatgttacacgagatgggaagaactgtgaagatatggatgaatgcagcataaggaacatgtgccttaatggaatgtgtatcaatgaagatggcagttttaaatgtatttgcaaacctggattccagctggcatcagatggacgttattgcaaagacattaacgagtgtgaaacccctgggatctgcatgaatgggcgttgcgtcaacactgatggctcctacagatgtgaatgcttccctggactggctgtgggtctggatggccgtgtgtgtgttgacacacacatgcggagcacatgctatggtggatacaagagaggccagtgtatcaaacctttgtttggtgctgtcactaaatctgaatgctgttgcgccagcactgagtatgcatttggggaaccttgccagccgtgtcctgcacagaattcagcggaatatcaggcactctgcagcagtgggccaggaatgacgtcagcaggcagtgatataaatgaatgtgcactagatcctgatatttgcccaaatggaatctgtgaaaaccttcgtgggacctataaatgtatatgcaattcaggatatgaagtggattcaactgggaaaaactgcgttgatattaatgaatgtgtactgaacagtctcctttgtgacaatggacaatgtagaaatactcctggaagttttgtctgtacctgccccaagggatttatctacaaacctgatctaaaaacatgtgaagacattgatgaatgcgaatcaagtccttgcattaatggagtctgcaagaacagcccaggctcttttatttgtgaatgttcttctgaaagtactttggatccaacaaaaaccatctgcatagaaaccatcaagggcacttgctggcagactgtcattgatgggcgatgtgagatcaacatcaatggagccaccttaaagtcccagtgctgctcctccctcggtgctgcgtggggaagcccgtgcaccctatgccaagttgatcccatatgtggtaaagggtactcaagaattaaaggaacacaatgtgaagatatagatgaatgtgaagtgttcccaggagtgtgtaaaaatggcctgtgtgttaacactagggggtcattcaagtgtcagtgtcccagtggaatgactttggatgccacaggaaggatctgtcttgatatccgcctggaaacctgcttcctgaggtacgaggacgaggagtgcaccctgcctattgctggccgccaccgcatggacgcctgctgctgctccgtcggggcagcctggggtactgaggaatgcgaggagtgtcccatgagaaatactcctgagtacgaggagctgtgtccgagaggacccggatttgccacaaaagaaattacaaatggaaagcctttcttcaaagatatcaatgagtgcaagatgatacccagcctctgcacccacggcaagtgcagaaacaccattggcagctttaagtgcaggtgtgacagcggctttgctcttgattctgaagaaaggaactgcacagacattgacgaatgccgcatatctcctgacctctgtggcagaggccagtgtgtgaacacccctggggactttgaatgcaagtgtgacgaaggctatgaaagtggattcatgatgatgaagaactgcatggatattgatgagtgtcagagagatcctctcctatgccgaggtggtgtttgccataacacagagggaagttaccgctgtgaatgcccgcctggccatcagctgtcccccaacatctccgcgtgtatcgacatcaatgaatgtgagctgagtgcacacctgtgccccaatggccgttgcgtgaacctcatagggaagtatcagtgtgcctgcaaccctggctaccattcaactcccgataggctattttgtgttgacattgatgaatgcagcataatgaatggtggttgtgaaaccttctgcacaaactctgaaggcagctatgaatgtagctgtcagccgggatttgcactaatgcctgaccagagatcatgcaccgacatcgatgagtgtgaagataatcccaatatctgtgatggtggtcagtgcacaaatatccctggagagtacaggtgcttgtgttatgatggattcatggcatctgaagacatgaagacttgtgtagatgtcaatgagtgtgacctgaatccaaatatctgcctaagtgggacctgtgaaaacacgaaaggctcatttatctgccactgtgatatgggctactccggcaaaaaaggaaaaactggctgtacagacatcaatgaatgtgaaattggagcacacaactgtggcaaacatgctgtatgtaccaatacagcaggaagcttcaaatgtagctgcagtcccgggtggattggagatggcattaagtgcactgatctggacgaatgttccaatggaacccatatgtgcagccagcatgcagactgcaagaataccatgggatcttaccgctgtctgtgcaaggaaggatacacaggtgatggcttcacttgtacagaccttgatgagtgctctgagaacctgaatctctgtggcaatggccagtgcctcaatgcaccaggaggataccgctgtgaatgcgacatgggcttcgtgcccagtgctgacgggaaagcctgtgaagatattgatgagtgctcccttccgaacatctgtgtctttggaacttgccacaacctccctggcctgttccgctgtgagtgtgagataggctacgaactggacagaagcggcgggaactgcacagatgtgaatgaatgcctggatccaaccacgtgcatcagtgggaactgtgtcaacactccaggcagctatatctgtgactgcccacctgattttgaactgaacccaactcgagttggctgtgttgatacccgctctggaaattgctatttggatattcgacctcgaggagacaatggagatacagcctgcagcaatgaaattggagttggtgtttccaaagcttcctgctgctgttctctgggtaaagcctggggtactccttgtgagatgtgtcctgctgtgaacacatccgagtacaaaattctttgtcctggaggggaaggtttccgaccaaatcctatcaccgttatattggaagatattgatgagtgccaggagctaccagggctgtgccaaggaggaaaatgtatcaacacctttgggagtttccagtgccgctgtccaaccggctactacctgaatgaagatacacgagtgtgtgatgatgtgaatgaatgtgagactcctggaatctgtggtccagggacatgttacaacaccgttggcaactacacctgtatctgtcctccagactacatgcaagtgaatgggggaaataattgcatggatatgagaagaagtttgtgctacagaaactactatgctgacaaccagacctgtgatggagaattgttattcaacatgaccaagaagatgtgctgctgttcctacaacattggccgggcgtggaacaagccctgtgaacagtgtcccatcccaagtacagatgagtttgctacactctgtggaagtcaaaggccaggctttgtcatcgacatttataccggtttacccgttgatattgatgagtgccgggagatcccaggggtctgtgaaaatggagtgtgtatcaacatggttggcagcttccgatgtgaatgtccagtgggattcttctataatgacaagttgttggtttgtgaagatattgacgagtgtcagaacggcccagtgtgccagcgcaacgccgaatgcatcaacactgcaggcagctaccgctgtgactgtaagcccggctaccgcttcacctccacaggacagtgcaatgatcgtaatgaatgtcaagaaatccccaatatatgcagtcatgggcagtgcattgacacagttggaagcttttattgcctttgccacactggttttaaaacaaatgatgaccaaaccatgtgcttggacataaatgaatgtgaaagagatgcctgtgggaatggaacttgccggaacacaattggttccttcaactgccgctgcaatcatggtttcatcctttctcacaacaatgactgtatagatgttgatgaatgtgcaagtggaaatgggaatctttgcagaaatggccaatgcattaatacagtggggtctttccagtgccagtgcaatgaaggctatgaggtggctccagatgggaggacctgtgtggatatcaatgaatgtcttctagaacccagaaaatgtgcaccaggtacctgtcaaaacttggatgggtcctacagatgcatttgcccacctggatacagtcttcaaaatgagaagtgtgaagatattgatgagtgtgtcgaagagccagaaatttgtgccctgggcacatgcagtaacactgaaggcagcttcaaatgtctgtgtccagaagggttttccttgtcctccagtggaagaaggtgccaagatttgcgaatgagctactgttatgcgaagtttgaaggaggaaagtgttcatcacccaaatccagaaatcactccaagcaggaatgctgctgtgccttgaagggagaaggctggggagacccctgcgagctctgccccacggaacctgatgaggccttccgccagatatgtccttatggaagtgggatcatcgtgggacctgatgattcagcagttgatatggacgaatgcaaagaacccgatgtctgtaaacatggacagtgcatcaatacagatggttcctatcgctgcgagtgtccctttggttatattctagcagggaatgaatgtgtagatactgatgaatgttctgttggcaatccttgtggaaatggaacctgcaagaatgtgattggaggttttgaatgcacctgcgaggagggatttgagcccggtccaatgatgacatgtgaagatataaatgaatgtgcccagaatcctctgctctgtgccttccgatgtgtgaacacttatgggtcatatgaatgcaaatgtcccgtgggatatgtgctcagagaagaccgtaggatgtgcaaagatgaggatgagtgtgaagagggaaaacatgactgtactgaaaaacaaatggaatgcaagaacctcattggcacatatatgtgcatctgtggacccgggtatcagcggagacctgatggagaaggctgtgtagatgagaatgaatgtcagacgaagccagggatctgtgagaatgggcgctgcctcaacacccgtgggagctacacctgtgagtgtaatgatgggtttaccgccagccccaaccaggacgagtgccttgacaatcgggaagggtactgcttcacagaggtgctacaaaacatgtgtcagatcggctccagcaacaggaaccccgtcaccaaatcggaatgctgctgtgacggagggagaggctggggtccccactgtgagatctgccctttccaggggactgtggctttcaagaaactctgtccccatggccgaggattcatgaccaatggagcagatatcgatgaatgcaaggttattcacgatgtttgccgaaatggggaatgtgtcaatgacagaggatcatatcattgcatttgtaaaactgggtacactccagatataactgggacttcctgtgtagatctgaacgagtgcaaccaggctcccaaaccctgcaattttatctgcaaaaacacagaagggagttaccagtgttcatgcccgaaaggctacattctgcaagaggatggaaggagctgcaaagatcttgatgagtgtgcaaccaagcaacacaactgccagttcctatgtgttaacaccattggcggcttcacatgcaaatgtcctcccggatttacccaacaccatacgtcctgcattgataacaatgaatgcacctctgacatcaatctgtgcgggtctaagggcatttgccagaacactcctggaagcttcacctgtgaatgccagcggggattctcacttgatcagaccggctccagctgtgaagacgtggacgagtgtgagggtaaccaccgctgccagcatggctgccagaacatcattgggggctacaggtgcagctgcccccagggctacctccagcactaccagtggaaccagtgtgttgatgaaaacgaatgcctcagcgctcacatctgcggaggagcctcctgtcacaacaccctggggagctacaagtgcatgtgtcccgccggcttccagtatgaacagttcagtggaggatgccaagacatcaatgaatgtggctctgcgcaggccccctgcagctatggctgttccaataccgagggcggttacctgtgtggctgtccacctggttacttccgcataggccaagggcactgtgtttctggaatgggcatgggccgaggaaacccagagccacctgtcagtggtgaaatggatgacaattcactctccccagaggcttgttacgagtgtaagatcaatggctaccccaaacggggcaggaaacggagaagcacaaacgaaactgatgcctccaatatcgaggatcagtctgagacagaagccaatgtgagtcttgcaagttgggatgttgagaagacagccatctttgctttcaatatttcccacgtcagtaacaaggttcgaatcctagaactccttccagctcttacaactctgacgaatcacaacagatacttgatcgaatctggaaatgaagatggcttctttaaaatcaaccaaaaggaagggatcagctacctccacttcacaaagaagaagccagtggctggaacctattcattacaaatcagtagtactccactttataaaaagaaagaacttaaccaactagaagacaaatatgacaaagactacctcagtggtgaactgggtgataatctgaagatgaaaatccaggttttgcttcattaa

SEQ ID NO: 20 - DNA, 8622 bp, Mus musculus
atgcggcgaggagggctgctggaggtcgcgctggcgttcgccctgctcctcgagtcctacacgagccatggggcggacgccaatttggaggctgggagcctgaaggagaccagagccaatcgggccaagagaagaggcggcggaggacacgatgcgctgaaaggacccaatgtctgtggatcacgttataatgcatactgttgtcctggatggaaaaccttacctggtggaaatcagtgtattgttcccatttgccggcattcctgtggggatggattctgctcgaggccaaatatgtgcacttgcccgtctggtcagatatctccttcctgtggctccagatccatccaacactgcagcatccgctgtatgaatgggggcagctgcagcgatgaccactgtctgtgccagaaagggtacatcggcactcactgtggacagcctgtctgtgaaagtggctgtctcaacggagggaggtgtgtggccccaaatcggtgtgcttgcacgtacggctttactggaccccagtgtgaaagagattacagaacaggcccatgttttactgtggtaagcaaccagatgtgccagggacagctcagcgggattgtctgcaccaaaacactttgctgtgccaccgtgggccgagcctggggccacccctgtgagatgtgtcctgcccagcctcacccctgccgccgcggcttcattcccaacatccgcactggagcttgtcaagatgtggatgaatgtcaggccatcccagggatgtgtcaaggaggaaattgcattaataccgttggatcttttgagtgcaaatgccctgctggacacaaatttaatgaagtgtcacaaaaatgtgaagatattgacgagtgcagcaccattcctggagtctgcgatggcggggaatgtacaaacactgtcagcagctacttctgcaaatgtccccctggtttttacacctctcctgatggcaccagatgcgtagatgttcgccctggttactgctacacagctctggcaaacgggcgctgctctaaccagctgccacagtccataaccaaaatgcagtgctgttgcgatcttggccggtgctggtctccaggggttactgttgctcccgagatgtgtcccatcaggtcaactgaggatttcaacaagctgtgctctgtccctctggtaattcccgggagaccagaatatcctcccccacccattggcccccttcctccagttcagcccgttcctcctggctatcctcctgggcctgtgattccagcccctcggccaccgccagaatatccatatccatctccgtctcgggaaccaccaagggtgctgcctttcaacgttactgactactgtcaactggtccgctatctctgtcaaaatgggcgctgcattccaactcccggtagctaccgctgcgagtgcaacaagggcttccagctggatatccgtggcgaatgcatcgacgtggatgagtgtgagaagaacccatgcactggtggcgagtgcatcaacaaccagggctcctacacctgtcactgcagagctggctaccagagcacactcaccagaactgagtgcagagacatagatgagtgtcttcagaatggccggatctgcaacaatggtcgctgtatcaacacagacggcagcttccactgcgtatgcaatgcgggctttcatgtcacgcgggacggaaagaactgtgaagatatggatgagtgcagcatccgaaacatgtgcctaaacggaatgtgtattaatgaagatggcagtttcaagtgtatttgcaaacctgggttccaactggcatcagatggccgctactgcaaagatatcaatgagtgtgagacacctgggatctgcatgaacggacgctgtgtgaacacggatggctcctacagatgcgaatgcttccccggattggctgtgggtctagacggacgtgtgtgtgttgacacacacatgcggagcacatgctatggaggatacaggagaggccagtgcgtgaagccgttgtttggtgctgttaccaaatcggaatgctgttgtgccagcactgagtatgcctttggggaaccctgccagccgtgtcctgcacagaattcagcggaatatcaggcactctgcagcagtggaccgggaatgacatcagcaggcactgatataaacgaatgtgcattagatcctgatatttgcccaaatggaatttgtgaaaatctccgtgggacctacaaatgtatatgcaactcgggatatgaagtagacataactgggaaaaactgtgtcgatattaatgagtgtgtgctgaacagtctactttgtgacaatggacaatgtcgaaacacacctggaagttttgtctgcacctgccccaaaggatttgtgtacaaacctgacctaaaaacctgtgaagacattgatgaatgtgaatcgagtccttgcattaatggagtctgcaagaacagccctggctccttcatttgtgaatgttctcctgaaagtactctggacccaacaaaaaccatctgcatagaaaccatcaagggcacttgctggcagactgtcatcgacgggcgctgtgagatcaacatcaacggagccaccttgaagtccgagtgctgctcctcccttggtgctgcgtgggggagcccgtgcaccatctgtcaacttgatcccatttgtggtaaagggttctcaagaattaaaggcacgcaatgtgaagatatcaatgagtgtgaagtgttcccgggagtatgcaagaacggcctgtgtgtcaactccaggggttcattcaagtgcgagtgtcccaatggaatgactttggatgctacaggaagaatctgtcttgacatccgcctggagacctgcttcctcaagtatgacgatgaagagtgcaccttgcccatcgctggccgccaccgaatggatgcctgctgctgctctgttggggcagcctggggaacggaagagtgtgaggagtgtccattgagaaacagccgggagtatgaggaactctgtccccgaggacctgggtttgccacaaaagacattacaaatgggaaacctttcttcaaagatatcaatgagtgcaagatgatacccagcctctgtacccacggcaagtgcaggaacaccattggcagcttcaagtgtaggtgtgacagtggctttgctctggattctgaagagaggaactgtacagacattgatgagtgccgcatatctcctgacctctgtggccgaggccagtgtgtgaacaccccgggggactttgaatgcaagtgtgatgaaggctatgaaagtggcttcatgatgatgaagaactgcatggatattgatgaatgtcagagagatcctctcctgtgtcgaggaggcatttgccacaacacagagggaagctatcgctgcgaatgtcctcctggtcaccaattgtccccaaacatctctgcatgcattgacatcaacgagtgtgagctgagtgcgaatctctgtccccatgggcgttgtgtgaacctcatagggaagtaccagtgtgcctgcaaccctggctaccaccccactcatgacaggctcttctgtgtcgatattgatgaatgcagcataatgaacggtggttgtgagaccttctgcacaaactctgacgggagctatgaatgtagctgtcagccaggcttcgcgctaatgccagaccagcgatcgtgcacagacattgatgagtgtgaagacaaccccaatatctgtgatggtggccagtgcacaaacatacctggggagtacaggtgcctgtgctatgatgggttcatggcatctgaagacatgaagacttgtgtggatgtcaatgagtgtgacctgaatccaaacatctgccttagtgggacctgtgaaaatactaaaggctcgttcatctgccactgtgatatgggatattcagggaagaaaggaaaaacgggctgtacagatatcaatgaatgtgagatcggagcacacaactgtggcagacatgctgtatgcacaaatacagccgggagcttcaagtgcagctgcagtcccggctggattggagacggcattaagtgcacagatctggatgaatgctctaatggaacccacatgtgcagccaacacgcggactgcaagaacaccatggggtcatatcgctgtctctgtaaggatggctatacaggggatggcttcacctgtacagacctcgacgagtgctccgagaacctgaacctctgtggcaatggccagtgcctcaacgcccctggcgggtaccgctgtgaatgcgacatgggcttcgtgcccagtgctgacgggaaggcctgtgaagatatcgatgagtgctcccttccaaacatctgtgtctttggaacttgccacaacctcccgggcctcttccgttgcgagtgtgagattggctatgaactggaccgaagtggtggaaactgcacagatgttaatgagtgtctggatcccaccacctgcatcagtggaaactgtgtcaacactcccggtagttacacatgcgattgtcctccggattttgagctgaatccaactcgtgtcggctgtgtcgatactcgctctggaaactgctatctggatatccgaccccggggagacaatggagatacagcctgcagcaatgaaattggagttggtgtctctaaggcttcctgctgttgttcactgggtaaagcttggggaaccccatgtgagctgtgtccttctgtgaacacatctgagtataaaattctttgccctggaggagaaggttttcgtccaaatcccatcaccgttatattggaagacatcgatgagtgccaggagcttccagggctgtgccaaggggggaagtgcatcaatacctttggcagcttccagtgtcgctgtccaactggttactacctgaatgaagacactcgagtgtgtgatgatgtgaacgaatgtgagactcctggaatctgtggtccggggacctgttacaacaccgttggcaactatacctgcatttgtcctccagactacatgcaagtgaacgggggaaataattgcatggacatgagaagaagtctatgctacagaaactattacgctgacaaccagacctgcgatggagaactcctgttcaacatgaccaagaagatgtgctgttgctcctacaacatcggcagagcctggaacaaaccctgtgaacagtgccccatcccaagcacagatgagtttgctaccctctgtgggagccagaggcccggcttcgtgattgacatttatacgggtttacccgtggatattgatgaatgccgggagatccctggggtctgtgaaaatggagtgtgcatcaacatggttggcagcttccggtgtgagtgtcccgtgggattcttctataacgacaagttactggtttgtgaagatatcgacgagtgtcagaatggccctgtgtgccagcgaaatgcggaatgcatcaacactgcaggcagctaccgctgtgactgtaagcccggctaccgccttacctccacaggtcaatgcaacgatcgaaacgagtgccaagaaatcccgaacatatgcagtcatggccagtgcatcgacaccgtgggaagcttctactgcctttgtcacactggcttcaaaacaaatgtggatcagaccatgtgcttagacataaatgagtgtgagagagacgcctgtgggaacgggacttgcagaaacacgattggctccttcaactgtcgctgtaaccatggcttcatactgtctcacaacaatgactgcatagatgttgatgagtgtgcaactggaaacgggaacctttgcagaaatggccagtgtgtcaataccgtgggctcctttcagtgcaggtgcaatgaaggctatgaggtggctccggacggcaggacctgtgtggatatcaacgagtgtgttctggatcctgggaaatgtgcacctggaacctgtcagaacctggatggctcctacagatgcatttgcccgcctgggtatagtctacagaatgacaagtgtgaagatattgatgagtgtgttgaagagccagaaatctgtgccttggggacctgcagcaacactgagggtagcttcaaatgtctgtgtccagaggggttctccctgtcctccactggaagaaggtgccaagatttgcgaatgagctactgctatgcgaagtttgaaggtgggaagtgttcatcacccaaatccagaaaccattccaagcaggagtgctgctgtgctttgaagggagaaggctggggagatccttgtgagttgtgccccactgagccagatgaggctttccgccagatctgcccctttggaagtgggatcattgtgggccctgatgactcagcagttgatatggacgaatgcaaagaacctgatgtctgtagacatgggcagtgcattaacacagacggctcctatcgatgcgagtgtccttttggttatattctggaagggaatgagtgtgtggataccgatgaatgctctgtgggcaatccttgtggaaatgggacctgcaagaatgtgattggaggttttgaatgtacctgtgaggaggggttcgagcctggcccaatgatgacttgtgaagatataaatgaatgtgcccagaatcctctgctctgcgccttccgctgtgtaaatacctacgggtcctatgaatgcaaatgccctgttggatacgttctccgagaagacaggaggatgtgtaaagatgaggatgagtgtgcagagggaaaacacgactgtactgagaagcaaatggagtgtaagaacctcattggtacctacatgtgcatctgcggccctgggtaccagcgcagacccgatggagagggctgcatagatgagaatgagtgtcagaccaagcccgggatctgtgagaatgggcgttgcctcaacaccctgggtagctacacttgtgagtgtaacgatggcttcacagccagccccactcaggatgagtgcttggacaaccgggaagggtactgcttttcggaggtcttgcaaaacatgtgccagattggctcaagcaacaggaaccccgtcaccaagtccgagtgctgctgtgatggagggagaggctggggaccccactgtgagatctgccctttcgagggcacagtggcttacaagaagctctgtccccacggccgaggattcatgaccaacggagcagatattgatgagtgcaaggttattcatgatgtttgccgaaatggggagtgtgtcaacgacagagggtcctatcactgcatctgtaaaactggctacactccggatataacagggaccgcctgtgtagatctgaatgaatgcaaccaggctcccaaaccctgcaattttatatgcaaaaacacagaagggagttaccagtgttcctgcccgaagggctacattctgcaagaggatggaaggagctgcaaagatcttgacgagtgtgcaaccaagcagcataactgtcagttcctgtgtgttaacaccatcggtggcttcacatgcaaatgccctcctgggtttacccagcatcacactgcctgcattgataacaatgagtgcacgtctgatatcaacctgtgtgggtccaagggtgtttgccagaacactccaggaagcttcacctgtgaatgccaacgggggttctcactcgatcagagtggtgccagctgtgaagatgtggacgagtgtgagggtaaccaccgctgtcaacatggctgccagaacatcatcggaggctataggtgtagctgcccccagggctacctccagcactaccaatggaaccagtgtgtagatgaaaacgagtgcctgagtgcacatgtctgtggaggagcctcctgccacaacaccctggggagttacaagtgcatgtgtcccaccggcttccagtacgaacagttcagtggaggctgccaagacatcaatgagtgtggctcatcccaggccccctgcagttacggttgctctaatactgagggtggctacctgtgtggctgtccaccaggatacttccggataggccaagggcattgtgtttctggaatgggcatgggccgaggcggcccagagccacctgccagcagcgagatggacgacaactcactgtccccagaggcctgctatgagtgtaagatcaacggctacccaaaacgaggccggaaacggagaagcacgaacgaaacggatgcctccgacatccaggacgggtctgagatggaagccaacgtgagcctcgccagctgggatgtggagaagccggctagctttgctttcaatatttcccatgtcaataacaaggtccgaatcctagagctcctgccggccctcacaactctgatgaaccacaacagatacttgattgaatctggaaatgaagatggcttctttaaaatcaaccagaaagaaggggtcagctacctccacttcacgaagaagaagccggtggctgggacctactccttacaaatcagcagcaccccactttataaaaagaaagaacttaaccagttagaagacagatatgacaaagactacctcagtggtgaactgggcgataacctgaagatgaaaattcagatcttgctgcattaa

SEQ ID NO: 21 - DNA, 8623 bp, Artificial Sequence
  Synthetic
atgcggcgaggagggctgctggaggtcgcgctggcgttcgccctgctcctcgagtcctacacgagccatggggcggacgccaatttggaggctgggagcctgaaggagaccagagccaatcgggccaagagaagaggcggcggaggacacgatgcgctgaaaggacccaatgtctgtggatcacgttataatgcatactgttgtcctggatggaaaaccttacctggtggaaatcagtgtattgttcccatttgccggcattcctgtggggatggattctgctcgaggccaaatatgtgcacttgcccgtctggtcagatatctccttcctgtggctccagatccatccaacactgcagcatccgctgtatgaatgggggcagctgcagcgatgaccactgtctgtgccagaaagggtacatcggcactcactgtggacagcctgtctgtgaaagtggctgtctcaacggagggaggtgtgtggccccaaatcggtgtgcttgcacgtacggctttactggaccccagtgtgaaagagattacagaacaggcccatgttttactgtggtaagcaaccagatgtgccagggacagctcagcgggattgtctgcaccaaaacactttgctgtgccaccgtgggccgagcctggggccacccctgtgagatgtgtcctgcccagcctcacccctgccgccgcggcttcattcccaacatccgcactggagcttgtcaagatgtggatgaatgtcaggccatcccagggatgtgtcaaggaggaaattgcattaataccgttggatcttttgagtgcaaatgccctgctggacacaaatttaatgaagtgtcacaaaaatgtgaagatattgacgagtgcagcaccattcctggagtctgcgatggcggggaatgtacaaacactgtcagcagctacttctgcaaatgtccccctggtttttacacctctcctgatggcaccagatgcgtagatgttcgccctggttactgctacacagctctggcaaacgggcgctgctctaaccagctgccacagtccataaccaaaatgcagtgctgttgcgatcttggccggtgctggtctccaggggttactgttgctcccgagatgtgtcccatcaggtcaactgaggatttcaacaagctgtgctctgtccctctggtaattcccgggagaccagaatatcctcccccacccattggcccccttcctccagttcagcccgttcctcctggctatcctcctgggcctgtgattccagcccctcggccaccgccagaatatccatatccatctccgtctcgggaaccaccaagggtgctgcctttcaacgttactgactactgtcaactggtccgctatctctgtcaaaatgggcgctgcattccaactcccggtagctaccgctgcgagtgcaacaagggcttccagctggatatccgtggcgaatgcatcgacgtggatgagtgtgagaagaacccatgcactggtggcgagtgcatcaacaaccagggctcctacacctgtcactgcagagctggctaccagagcacactcaccagaactgagtgcagagacatagatgagtgtcttcagaatggccggatctgcaacaatggtcgctgtatcaacacagacggcagcttccactgcgtatgcaatgcgggctttcatgtcacgcgggacggaaagaactgtgaagatatggatgagtgcagcatccgaaacatgtgcctaaacggaatgtgtattaatgaagatggcagtttcaagtgtatttgcaaacctgggttccaactggcatcagatggccgctactgcaaagatatcaatgagtgtgagacacctgggatctgcatgaacggacgctgtgtgaacacggatggctcctacagatgcgaatgcttccccggattggctgtgggtctagacggacgtgtgtgtgttgacacacacatgcggagcacatgctatggaggatacaggagaggccagtgcgtgaagccgttgtttggtgctgttaccaaatcggaatgctgttgtgccagcactgagtatgcctttggggaaccctgccagccgtgtcctgcacagaattcagcggaatatcaggcactctgcagcagtggaccgggaatgacatcagcaggcactgatataaacgaatgtgcattagatcctgatatttgcccaaatggaatttgtgaaaatctccgtgggacctacaaatgtatatgcaactcgggatatgaagtagacataactgggaaaaactgtgtcgatattaatgagtgtgtgctgaacagtctactttgtgacaatggacaatgtcgaaacacacctggaagttttgtctgcacctgccccaaaggatttgtgtacaaacctgacctaaaaacctgtgaagacattgatgaatgtgaatcgagtccttgcattaatggagtctgcaagaacagccctggctccttcatttgtgaatgttctcctgaaagtactctggacccaacaaaaaccatctgcatagaaaccatcaagggcacttgctggcagactgtcatcgacgggcgctgtgagatcaacatcaacggagccaccttgaagtccgagtgctgctcctcccttggtgctgcgtgggggagcccgtgcaccatctgtcaacttgatcccatttgtggtaaagggttctcaagaattaaaggcacgcaatgtgaagatatcaatgagtgtgaagtgttcccgggagtatgcaagaacggcctgtgtgtcaactccaggggttcattcaagtgcgagtgtcccaatggaatgactttggatgctacaggaagaatctgtcttgacatccgcctggagacctgcttcctcaagtatgacgatgaagagtgcaccttgcccatcgctggccgccaccgaatggatgcctgctgctgctctgttggggcagcctggggaacggaagagtgtgaggagtgtccattgagaaacagccgggagtatgaggaactctgtccccgaggacctgggtttgccacaaaagacattacaaatgggaaacctttcttcaaagatatcaatgagtgcaagatgatacccagcctctgtacccacggcaagtgcaggaacaccattggcagcttcaagtgtaggtgtgacagtggctttgctctggattctgaagagaggaactgtacagacattgatgagtgccgcatatctcctgacctctgtggccgaggccagtgtgtgaacaccccgggggactttgaatgcaagtgtgatgaaggctatgaaagtggcttcatgatgatgaagaactgcatggatattgatgaatgtcagagagatcctctcctgtgtcgaggaggcatttgccacaacacagagggaagctatcgctgcgaatgtcctcctggtcaccaattgtccccaaacatctctgcatgcattgacatcaacgagtgtgagctgagtgcgaatctctgtccccatgggcgttgtgtgaacctcatagggaagtaccagtgtgcctgcaaccctggctaccaccccactcatgacaggctcttctgtgtcgatattgatgaatgcagcataatgaacggtggttgtgagaccttctgcacaaactctgacgggagctatgaatgtagctgtcagccaggcttcgcgctaatgccagaccagcgatcgtgcacagacattgatgagtgtgaagacaaccccaatatctgtgatggtggccagtgcacaaacatacctggggagtacaggtgcctgtgctatgatgggttcatggcatctgaagacatgaagacttgtgtggatgtcaatgagtgtgacctgaatccaaacatctgccttagtgggacctgtgaaaatactaaaggctcgttcatctgccactgtgatatgggatattcagggaagaaaggaaaaacgggctgtacagatatcaatgaatgtgagatcggagcacacaactgtggcagacatgctgtatgcacaaatacagccgggagcttcaagtgcagctgcagtcccggctggattggagacggcattaagtgcacagatctggatgaatgctctaatggaacccacatgtgcagccaacacgcggactgcaagaacaccatggggtcatatcgctgtctctgtaaggatggctatacaggggatggcttcacctgtacagacctcgacgagtgctccgagaacctgaacctctgtggcaatggccagtgcctcaacgcccctggcgggtaccgctgtgaatgcgacatgggcttcgtgcccagtgctgacgggaaggcctgtgaagatatcgatgagtgctcccttccaaacatctgtgtctttggaacttgccacaacctcccgggcctcttccgttgcgagtgtgagattggctatgaactggaccgaagtggtggaaactgcacagatgttaatgagtgtctggatcccaccacctgcatcagtggaaactgtgtcaacactcccggtagttacacatgcgattgtcctccggattttgagctgaatccaactcgtgtcggctgtgtcgatactcgctctggaaactgctatctggatatccgaccccggggagacaatggagatacagcctgcagcaatgaaattggagttggtgtctctaaggcttcctgctgttgttcactgggtaaagcttggggaaccccatgtgagctgtgtccttctgtgaacacatctgagtataaaattctttgccctggaggagaaggttttcgtccaaatcccatcaccgttatattggaagacatcgatgagtgccaggagcttccagggctgtgccaaggggggaagtgcatcaatacctttggcagcttccagtgtcgctgtccaactggttactacctgaatgaagacactcgagtgtgtgatgatgtgaacgaatgtgagactcctggaatctgtggtccggggacctgttacaacaccgttggcaactatacctgcatttgtcctccagactacatgcaagtgaacgggggaaataattgcatggacatgagaagaagtctatgctacagaaactattacgctgacaaccagacctgcgatggagaactcctgttcaacatgaccaagaagatgtgctgttgctcctacaacatcggcagagcctggaacaaaccctgtgaacagtgccccatcccaagcacagatgagtttgctaccctctgtgggagccagaggcccggcttcgtgattgacatttatacgggtttacccgtggatattgatgaatgccgggagatccctggggtctgtgaaaatggagtgtgcatcaacatggttggcagcttccggtgtgagtgtcccgtgggattcttctataacgacaagttactggtttgtgaagatatcgacgagtgtcagaatggccctgtgtgccagcgaaatgcggaatgcatcaacactgcaggcagctaccgctgtgactgtaagcccggctaccgccttacctccacaggtcaatgcaacgatcgaaacgagtgccaagaaatcccgaacatatgcagtcatggccagtgcatcgacaccgtgggaagcttctactgcctttgtcacactggcttcaaaacaaatgtggatcagaccatgtgcttagacataaatgagtgtgagagagacgcctgtgggaacgggacttgcagaaacacgattggctccttcaactgtcgctgtaaccatggcttcatactgtctcacaacaatgactgcatagatgttgatgagtgtgcaactggaaacgggaacctttgcagaaatggccagtgtgtcaataccgtgggctcctttcagtgcaggtgcaatgaaggctatgaggtggctccggacggcaggacctgtgtggatatcaacgagtgtgttctggatcctgggaaatgtgcacctggaacctgtcagaacctggatggctcctacagatgcatttgcccgcctgggtatagtctacagaatgacaagtgtgaagatattgatgagtgtgttgaagagccagaaatctgtgccttggggacctgcagcaacactgagggtagcttcaaatgtctgtgtccagaggggttctccctgtcctccactggaagaaggtgccaagatttgcgaatgagctactgctatgcgaagtttgaaggtgggaagtgttcatcacccaaatccagaaaccattccaagcaggagtgctgctgtgctttgaagggagaaggctggggagatccttgtgagttgtgccccactgagccagatgaggctttccgccagatctgcccctttggaagtgggatcattgtgggccctgatgactcagcagttgatatggacgaatgcaaagaacctgatgtctgtagacatgggcagtgcattaacacagacggctcctatcgatgcgagtgtccttttggttatattctggaagggaatgagtgtgtggataccgatgaatgctctgtgggcaatccttgtggaaatgggacctgcaagaatgtgattggaggttttgaatgtacctgtgaggaggggttcgagcctggcccaatgatgacttgtgaagatataaatgaatgtgcccagaatcctctgctctgcgccttccgctgtgtaaatacctacgggtcctatgaatgcaaatgccctgttggatacgttctccgagaagacaggaggatgtgtaaagatgaggatgagtgtgcagagggaaaacacgactgtactgagaagcaaatggagtgtaagaacctcattggtacctacatgtgcatctgcggccctgggtaccagcgcagacccgatggagagggctgcatagatgagaatgagtgtcagaccaagcccgggatctgtgagaatgggcgttgcctcaacaccctgggtagctacacttgtgagtgtaacgatggcttcacagccagccccactcaggatgagtgcttggacaaccgggaagggtactgcttttcggaggtcttgcaaaacatgtgccagattggctcaagcaacaggaaccccgtcaccaagtccgagtgctgctgtgatggagggagaggctggggaccccactgtgagatctgccctttcgagggcacagtggcttacaagaagctctgtccccacggccgaggattcatgaccaacggagcagatattgatgagtgcaaggttattcatgatgtttgccgaaatggggagtgtgtcaacgacagagggtcctatcactgcatctgtaaaactggctacactccggatataacagggaccgcctgtgtagatctgaatgaatgcaaccaggctcccaaaccctgcaattttatatgcaaaaacacagaagggagttaccagtgttcctgcccgaagggctacattctgcaagaggatggaaggagctgcaaagatcttgacgagtgtgcaaccaagcagcataactgtcagttcctgtgtgttaacaccatcggtggcttcacatgcaaatgccctcctgggtttacccagcatcacactgcctgcattgataacaatgagtgcacgtctgatatcaacctgtgtgggtccaagggtgtttgccagaacactccaggaagcttcacctgtgaatgccaacgggggttctcactcgatcagagtggtgccagctgtgaagatgtggacgagtgtgagggtaaccaccgctgtcaacatggctgccagaacatcatcggaggctataggtgtagctgcccccagggctacctccagcactaccaatggaaccagtgtgtagatgaaaacgagtgcctgagtgcacatgtctgtggaggagcctcctgccacaacaccctggggagttacaagtgcatgtgtcccaccggcttccagtacgaacagttcagtggaggctgccaagacatcaatgagtgtggctcatcccaggccccctgcagttacggttgctctaatactgagggtggctacctgtgtggctgtccaccaggatacttccggataggccaagggcattgtgtttctggaatgggcatgggccgaggcggcccagagccacctgccagcagcgagatggacgacaactcactgtccccagaggcctgctatgagtgtaagatcaacggctacccaaaacgaggccggaaacggagaagcacgaacgaaaactgatgcctccgacatccaggacgggtctgagatggaagccaacgtgagcctcgccagctgggatgtggagaagccggctagctttgctttcaatatttcccatgtcaataacaaggtccgaatcctagagctcctgccggccctcacaactctgatgaaccacaacagatacttgattgaatctggaaatgaagatggcttctttaaaatcaaccagaaagaaggggtcagctacctccacttcacgaagaagaagccggtggctgggacctactccttacaaatcagcagcaccccactttataaaaagaaagaacttaaccagttagaagacagatatgacaaagactacctcagtggtgaactgggcgataacctgaagatgaaaattcagatcttgctgcattaa

SEQ ID NO: 22 - DNA, 8647 bp, Artificial Sequence
  Synthetic
atgcggcgaggagggctgctggaggtcgcgctggcgttcgccctgctcctcgagtcctacacgagccatggggcggacgccaatttggaggctgggagcctgaaggagaccagagccaatcgggccaagagaagaggcggcggaggacacgatgcgctgaaaggacccaatgtctgtggatcacgttataatgcatactgttgtcctggatggaaaaccttacctggtggaaatcagtgtattgttcccatttgccggcattcctgtggggatggattctgctcgaggccaaatatgtgcacttgcccgtctggtcagatatctccttcctgtggctccagatccatccaacactgcagcatccgctgtatgaatgggggcagctgcagcgatgaccactgtctgtgccagaaagggtacatcggcactcactgtggacagcctgtctgtgaaagtggctgtctcaacggagggaggtgtgtggccccaaatcggtgtgcttgcacgtacggctttactggaccccagtgtgaaagagattacagaacaggcccatgttttactgtggtaagcaaccagatgtgccagggacagctcagcgggattgtctgcaccaaaacactttgctgtgccaccgtgggccgagcctggggccacccctgtgagatgtgtcctgcccagcctcacccctgccgccgcggcttcattcccaacatccgcactggagcttgtcaagatgtggatgaatgtcaggccatcccagggatgtgtcaaggaggaaattgcattaataccgttggatcttttgagtgcaaatgccctgctggacacaaatttaatgaagtgtcacaaaaatgtgaagatattgacgagtgcagcaccattcctggagtctgcgatggcggggaatgtacaaacactgtcagcagctacttctgcaaatgtccccctggtttttacacctctcctgatggcaccagatgcgtagatgttcgccctggttactgctacacagctctggcaaacgggcgctgctctaaccagctgccacagtccataaccaaaatgcagtgctgttgcgatcttggccggtgctggtctccaggggttactgttgctcccgagatgtgtcccatcaggtcaactgaggatttcaacaagctgtgctctgtccctctggtaattcccgggagaccagaatatcctcccccacccattggcccccttcctccagttcagcccgttcctcctggctatcctcctgggcctgtgattccagcccctcggccaccgccagaatatccatatccatctccgtctcgggaaccaccaagggtgctgcctttcaacgttactgactactgtcaactggtccgctatctctgtcaaaatgggcgctgcattccaactcccggtagctaccgctgcgagtgcaacaagggcttccagctggatatccgtggcgaatgcatcgacgtggatgagtgtgagaagaacccatgcactggtggcgagtgcatcaacaaccagggctcctacacctgtcactgcagagctggctaccagagcacactcaccagaactgagtgcagagacatagatgagtgtcttcagaatggccggatctgcaacaatggtcgctgtatcaacacagacggcagcttccactgcgtatgcaatgcgggctttcatgtcacgcgggacggaaagaactgtgaagatatggatgagtgcagcatccgaaacatgtgcctaaacggaatgtgtattaatgaagatggcagtttcaagtgtatttgcaaacctgggttccaactggcatcagatggccgctactgcaaagatatcaatgagtgtgagacacctgggatctgcatgaacggacgctgtgtgaacacggatggctcctacagatgcgaatgcttccccggattggctgtgggtctagacggacgtgtgtgtgttgacacacacatgcggagcacatgctatggaggatacaggagaggccagtgcgtgaagccgttgtttggtgctgttaccaaatcggaatgctgttgtgccagcactgagtatgcctttggggaaccctgccagccgtgtcctgcacagaattcagcggaatatcaggcactctgcagcagtggaccgggaatgacatcagcaggcactgatataaacgaatgtgcattagatcctgatatttgcccaaatggaatttgtgaaaatctccgtgggacctacaaatgtatatgcaactcgggatatgaagtagacataactgggaaaaactgtgtcgatattaatgagtgtgtgctgaacagtctactttgtgacaatggacaatgtcgaaacacacctggaagttttgtctgcacctgccccaaaggatttgtgtacaaacctgacctaaaaacctgtgaagacattgatgaatgtgaatcgagtccttgcattaatggagtctgcaagaacagccctggctccttcatttgtgaatgttctcctgaaagtactctggacccaacaaaaaccatctgcatagaaaccatcaagggcacttgctggcagactgtcatcgacgggcgctgtgagatcaacatcaacggagccaccttgaagtccgagtgctgctcctcccttggtgctgcgtgggggagcccgtgcaccatctgtcaacttgatcccatttgtggtaaagggttctcaagaattaaaggcacgcaatgtgaagatatcaatgagtgtgaagtgttcccgggagtatgcaagaacggcctgtgtgtcaactccaggggttcattcaagtgcgagtgtcccaatggaatgactttggatgctacaggaagaatctgtcttgacatccgcctggagacctgcttcctcaagtatgacgatgaagagtgcaccttgcccatcgctggccgccaccgaatggatgcctgctgctgctctgttggggcagcctggggaacggaagagtgtgaggagtgtccattgagaaacagccgggagtatgaggaactctgtccccgaggacctgggtttgccacaaaagacattacaaatgggaaacctttcttcaaagatatcaatgagtgcaagatgatacccagcctctgtacccacggcaagtgcaggaacaccattggcagcttcaagtgtaggtgtgacagtggctttgctctggattctgaagagaggaactgtacagacattgatgagtgccgcatatctcctgacctctgtggccgaggccagtgtgtgaacaccccgggggactttgaatgcaagtgtgatgaaggctatgaaagtggcttcatgatgatgaagaactgcatggatattgatgaatgtcagagagatcctctcctgtgtcgaggaggcatttgccacaacacagagggaagctatcgctgcgaatgtcctcctggtcaccaattgtccccaaacatctctgcatgcattgacatcaacgagtgtgagctgagtgcgaatctctgtccccatgggcgttgtgtgaacctcatagggaagtaccagtgtgcctgcaaccctggctaccaccccactcatgacaggctcttctgtgtcgatattgatgaatgcagcataatgaacggtggttgtgagaccttctgcacaaactctgacgggagctatgaatgtagctgtcagccaggcttcgcgctaatgccagaccagcgatcgtgcacagacattgatgagtgtgaagacaaccccaatatctgtgatggtggccagtgcacaaacatacctggggagtacaggtgcctgtgctatgatgggttcatggcatctgaagacatgaagacttgtgtggatgtcaatgagtgtgacctgaatccaaacatctgccttagtgggacctgtgaaaatactaaaggctcgttcatctgccactgtgatatgggatattcagggaagaaaggaaaaacgggctgtacagatatcaatgaatgtgagatcggagcacacaactgtggcagacatgctgtatgcacaaatacagccgggagcttcaagtgcagctgcagtcccggctggattggagacggcattaagtgcacagatctggatgaatgctctaatggaacccacatgtgcagccaacacgcggactgcaagaacaccatggggtcatatcgctgtctctgtaaggatggctatacaggggatggcttcacctgtacagacctcgacgagtgctccgagaacctgaacctctgtggcaatggccagtgcctcaacgcccctggcgggtaccgctgtgaatgcgacatgggcttcgtgcccagtgctgacgggaaggcctgtgaagatatcgatgagtgctcccttccaaacatctgtgtctttggaacttgccacaacctcccgggcctcttccgttgcgagtgtgagattggctatgaactggaccgaagtggtggaaactgcacagatgttaatgagtgtctggatcccaccacctgcatcagtggaaactgtgtcaacactcccggtagttacacatgcgattgtcctccggattttgagctgaatccaactcgtgtcggctgtgtcgatactcgctctggaaactgctatctggatatccgaccccggggagacaatggagatacagcctgcagcaatgaaattggagttggtgtctctaaggcttcctgctgttgttcactgggtaaagcttggggaaccccatgtgagctgtgtccttctgtgaacacatctgagtataaaattctttgccctggaggagaaggttttcgtccaaatcccatcaccgttatattggaagacatcgatgagtgccaggagcttccagggctgtgccaaggggggaagtgcatcaatacctttggcagcttccagtgtcgctgtccaactggttactacctgaatgaagacactcgagtgtgtgatgatgtgaacgaatgtgagactcctggaatctgtggtccggggacctgttacaacaccgttggcaactatacctgcatttgtcctccagactacatgcaagtgaacgggggaaataattgcatggacatgagaagaagtctatgctacagaaactattacgctgacaaccagacctgcgatggagaactcctgttcaacatgaccaagaagatgtgctgttgctcctacaacatcggcagagcctggaacaaaccctgtgaacagtgccccatcccaagcacagatgagtttgctaccctctgtgggagccagaggcccggcttcgtgattgacatttatacgggtttacccgtggatattgatgaatgccgggagatccctggggtctgtgaaaatggagtgtgcatcaacatggttggcagcttccggtgtgagtgtcccgtgggattcttctataacgacaagttactggtttgtgaagatatcgacgagtgtcagaatggccctgtgtgccagcgaaatgcggaatgcatcaacactgcaggcagctaccgctgtgactgtaagcccggctaccgccttacctccacaggtcaatgcaacgatcgaaacgagtgccaagaaatcccgaacatatgcagtcatggccagtgcatcgacaccgtgggaagcttctactgcctttgtcacactggcttcaaaacaaatgtggatcagaccatgtgcttagacataaatgagtgtgagagagacgcctgtgggaacgggacttgcagaaacacgattggctccttcaactgtcgctgtaaccatggcttcatactgtctcacaacaatgactgcatagatgttgatgagtgtgcaactggaaacgggaacctttgcagaaatggccagtgtgtcaataccgtgggctcctttcagtgcaggtgcaatgaaggctatgaggtggctccggacggcaggacctgtgtggatatcaacgagtgtgttctggatcctgggaaatgtgcacctggaacctgtcagaacctggatggctcctacagatgcatttgcccgcctgggtatagtctacagaatgacaagtgtgaagatattgatgagtgtgttgaagagccagaaatctgtgccttggggacctgcagcaacactgagggtagcttcaaatgtctgtgtccagaggggttctccctgtcctccactggaagaaggtgccaagatttgcgaatgagctactgctatgcgaagtttgaaggtgggaagtgttcatcacccaaatccagaaaccattccaagcaggagtgctgctgtgctttgaagggagaaggctggggagatccttgtgagttgtgccccactgagccagatgaggctttccgccagatctgcccctttggaagtgggatcattgtgggccctgatgactcagcagttgatatggacgaatgcaaagaacctgatgtctgtagacatgggcagtgcattaacacagacggctcctatcgatgcgagtgtccttttggttatattctggaagggaatgagtgtgtggataccgatgaatgctctgtgggcaatccttgtggaaatgggacctgcaagaatgtgattggaggttttgaatgtacctgtgaggaggggttcgagcctggcccaatgatgacttgtgaagatataaatgaatgtgcccagaatcctctgctctgcgccttccgctgtgtaaatacctacgggtcctatgaatgcaaatgccctgttggatacgttctccgagaagacaggaggatgtgtaaagatgaggatgagtgtgcagagggaaaacacgactgtactgagaagcaaatggagtgtaagaacctcattggtacctacatgtgcatctgcggccctgggtaccagcgcagacccgatggagagggctgcatagatgagaatgagtgtcagaccaagcccgggatctgtgagaatgggcgttgcctcaacaccctgggtagctacacttgtgagtgtaacgatggcttcacagccagccccactcaggatgagtgcttggacaaccgggaagggtactgcttttcggaggtcttgcaaaacatgtgccagattggctcaagcaacaggaaccccgtcaccaagtccgagtgctgctgtgatggagggagaggctggggaccccactgtgagatctgccctttcgagggcacagtggcttacaagaagctctgtccccacggccgaggattcatgaccaacggagcagatattgatgagtgcaaggttattcatgatgtttgccgaaatggggagtgtgtcaacgacagagggtcctatcactgcatctgtaaaactggctacactccggatataacagggaccgcctgtgtagatctgaatgaatgcaaccaggctcccaaaccctgcaattttatatgcaaaaacacagaagggagttaccagtgttcctgcccgaagggctacattctgcaagaggatggaaggagctgcaaagatcttgacgagtgtgcaaccaagcagcataactgtcagttcctgtgtgttaacaccatcggtggcttcacatgcaaatgccctcctgggtttacccagcatcacactgcctgcattgataacaatgagtgcacgtctgatatcaacctgtgtgggtccaagggtgtttgccagaacactccaggaagcttcacctgtgaatgccaacgggggttctcactcgatcagagtggtgccagctgtgaagatgtggacgagtgtgagggtaaccaccgctgtcaacatggctgccagaacatcatcggaggctataggtgtagctgcccccagggctacctccagcactaccaatggaaccagtgtgtagatgaaaacgagtgcctgagtgcacatgtctgtggaggagcctcctgccacaacaccctggggagttacaagtgcatgtgtcccaccggcttccagtacgaacagttcagtggaggctgccaagacatcaatgagtgtggctcatcccaggccccctgcagttacggttgctctaatactgagggtggctacctgtgtggctgtccaccaggatacttccggataggccaagggcattgtgtttctggaatgggcatgggccgaggcggcccagagccacctgccagcagcgagatggacgacaactcactgtccccagaggcctgctatgagtgtaagatcaacggctacccaaaggcggcccagagccacctgccagcaacgaggccggaaacggagaagcacgaacgaaacggatgcctccgacatccaggacgggtctgagatggaagccaacgtgagcctcgccagctgggatgtggagaagccggctagctttgctttcaatatttcccatgtcaataacaaggtccgaatcctagagctcctgccggccctcacaactctgatgaaccacaacagatacttgattgaatctggaaatgaagatggcttctttaaaatcaaccagaaagaaggggtcagctacctccacttcacgaagaagaagccggtggctgggacctactccttacaaatcagcagcaccccactttataaaaagaaagaacttaaccagttagaagacagatatgacaaagactacctcagtggtgaactgggcgataacctgaagatgaaaattcagatcttgctgcattaa

SEQ ID NO: 23 - DNA, 8620 bp, Artificial Sequence
  Synthetic
atgcggcgaggagggctgctggaggtcgcgctggcgttcgccctgctcctcgagtcctacacgagccatggggcggacgccaatttggaggctgggagcctgaaggagaccagagccaatcgggccaagagaagaggcggcggaggacacgatgcgctgaaaggacccaatgtctgtggatcacgttataatgcatactgttgtcctggatggaaaaccttacctggtggaaatcagtgtattgttcccatttgccggcattcctgtggggatggattctgctcgaggccaaatatgtgcacttgcccgtctggtcagatatctccttcctgtggctccagatccatccaacactgcagcatccgctgtatgaatgggggcagctgcagcgatgaccactgtctgtgccagaaagggtacatcggcactcactgtggacagcctgtctgtgaaagtggctgtctcaacggagggaggtgtgtggccccaaatcggtgtgcttgcacgtacggctttactggaccccagtgtgaaagagattacagaacaggcccatgttttactgtggtaagcaaccagatgtgccagggacagctcagcgggattgtctgcaccaaaacactttgctgtgccaccgtgggccgagcctggggccacccctgtgagatgtgtcctgcccagcctcacccctgccgccgcggcttcattcccaacatccgcactggagcttgtcaagatgtggatgaatgtcaggccatcccagggatgtgtcaaggaggaaattgcattaataccgttggatcttttgagtgcaaatgccctgctggacacaaatttaatgaagtgtcacaaaaatgtgaagatattgacgagtgcagcaccattcctggagtctgcgatggcggggaatgtacaaacactgtcagcagctacttctgcaaatgtccccctggtttttacacctctcctgatggcaccagatgcgtagatgttcgccctggttactgctacacagctctggcaaacgggcgctgctctaaccagctgccacagtccataaccaaaatgcagtgctgttgcgatcttggccggtgctggtctccaggggttactgttgctcccgagatgtgtcccatcaggtcaactgaggatttcaacaagctgtgctctgtccctctggtaattcccgggagaccagaatatcctcccccacccattggcccccttcctccagttcagcccgttcctcctggctatcctcctgggcctgtgattccagcccctcggccaccgccagaatatccatatccatctccgtctcgggaaccaccaagggtgctgcctttcaacgttactgactactgtcaactggtccgctatctctgtcaaaatgggcgctgcattccaactcccggtagctaccgctgcgagtgcaacaagggcttccagctggatatccgtggcgaatgcatcgacgtggatgagtgtgagaagaacccatgcactggtggcgagtgcatcaacaaccagggctcctacacctgtcactgcagagctggctaccagagcacactcaccagaactgagtgcagagacatagatgagtgtcttcagaatggccggatctgcaacaatggtcgctgtatcaacacagacggcagcttccactgcgtatgcaatgcgggctttcatgtcacgcgggacggaaagaactgtgaagatatggatgagtgcagcatccgaaacatgtgcctaaacggaatgtgtattaatgaagatggcagtttcaagtgtatttgcaaacctgggttccaactggcatcagatggccgctactgcaaagatatcaatgagtgtgagacacctgggatctgcatgaacggacgctgtgtgaacacggatggctcctacagatgcgaatgcttccccggattggctgtgggtctagacggacgtgtgtgtgttgacacacacatgcggagcacatgctatggaggatacaggagaggccagtgcgtgaagccgttgtttggtgctgttaccaaatcggaatgctgttgtgccagcactgagtatgcctttggggaaccctgccagccgtgtcctgcacagaattcagcggaatatcaggcactctgcagcagtggaccgggaatgacatcagcaggcactgatataaacgaatgtgcattagatcctgatatttgcccaaatggaatttgtgaaaatctccgtgggacctacaaatgtatatgcaactcgggatatgaagtagacataactgggaaaaactgtgtcgatattaatgagtgtgtgctgaacagtctactttgtgacaatggacaatgtcgaaacacacctggaagttttgtctgcacctgccccaaaggatttgtgtacaaacctgacctaaaaacctgtgaagacattgatgaatgtgaatcgagtccttgcattaatggagtctgcaagaacagccctggctccttcatttgtgaatgttctcctgaaagtactctggacccaacaaaaaccatctgcatagaaaccatcaagggcacttgctggcagactgtcatcgacgggcgctgtgagatcaacatcaacggagccaccttgaagtccgagtgctgctcctcccttggtgctgcgtgggggagcccgtgcaccatctgtcaacttgatcccatttgtggtaaagggttctcaagaattaaaggcacgcaatgtgaagatatcaatgagtgtgaagtgttcccgggagtatgcaagaacggcctgtgtgtcaactccaggggttcattcaagtgcgagtgtcccaatggaatgactttggatgctacaggaagaatctgtcttgacatccgcctggagacctgcttcctcaagtatgacgatgaagagtgcaccttgcccatcgctggccgccaccgaatggatgcctgctgctgctctgttggggcagcctggggaacggaagagtgtgaggagtgtccattgagaaacagccgggagtatgaggaactctgtccccgaggacctgggtttgccacaaaagacattacaaatgggaaacctttcttcaaagatatcaatgagtgcaagatgatacccagcctctgtacccacggcaagtgcaggaacaccattggcagcttcaagtgtaggtgtgacagtggctttgctctggattctgaagagaggaactgtacagacattgatgagtgccgcatatctcctgacctctgtggccgaggccagtgtgtgaacaccccgggggactttgaatgcaagtgtgatgaaggctatgaaagtggcttcatgatgatgaagaactgcatggatattgatgaatgtcagagagatcctctcctgtgtcgaggaggcatttgccacaacacagagggaagctatcgctgcgaatgtcctcctggtcaccaattgtccccaaacatctctgcatgcattgacatcaacgagtgtgagctgagtgcgaatctctgtccccatgggcgttgtgtgaacctcatagggaagtaccagtgtgcctgcaaccctggctaccaccccactcatgacaggctcttctgtgtcgatattgatgaatgcagcataatgaacggtggttgtgagaccttctgcacaaactctgacgggagctatgaatgtagctgtcagccaggcttcgcgctaatgccagaccagcgatcgtgcacagacattgatgagtgtgaagacaaccccaatatctgtgatggtggccagtgcacaaacatacctggggagtacaggtgcctgtgctatgatgggttcatggcatctgaagacatgaagacttgtgtggatgtcaatgagtgtgacctgaatccaaacatctgccttagtgggacctgtgaaaatactaaaggctcgttcatctgccactgtgatatgggatattcagggaagaaaggaaaaacgggctgtacagatatcaatgaatgtgagatcggagcacacaactgtggcagacatgctgtatgcacaaatacagccgggagcttcaagtgcagctgcagtcccggctggattggagacggcattaagtgcacagatctggatgaatgctctaatggaacccacatgtgcagccaacacgcggactgcaagaacaccatggggtcatatcgctgtctctgtaaggatggctatacaggggatggcttcacctgtacagacctcgacgagtgctccgagaacctgaacctctgtggcaatggccagtgcctcaacgcccctggcgggtaccgctgtgaatgcgacatgggcttcgtgcccagtgctgacgggaaggcctgtgaagatatcgatgagtgctcccttccaaacatctgtgtctttggaacttgccacaacctcccgggcctcttccgttgcgagtgtgagattggctatgaactggaccgaagtggtggaaactgcacagatgttaatgagtgtctggatcccaccacctgcatcagtggaaactgtgtcaacactcccggtagttacacatgcgattgtcctccggattttgagctgaatccaactcgtgtcggctgtgtcgatactcgctctggaaactgctatctggatatccgaccccggggagacaatggagatacagcctgcagcaatgaaattggagttggtgtctctaaggcttcctgctgttgttcactgggtaaagcttggggaaccccatgtgagctgtgtccttctgtgaacacatctgagtataaaattctttgccctggaggagaaggttttcgtccaaatcccatcaccgttatattggaagacatcgatgagtgccaggagcttccagggctgtgccaaggggggaagtgcatcaatacctttggcagcttccagtgtcgctgtccaactggttactacctgaatgaagacactcgagtgtgtgatgatgtgaacgaatgtgagactcctggaatctgtggtccggggacctgttacaacaccgttggcaactatacctgcatttgtcctccagactacatgcaagtgaacgggggaaataattgcatggacatgagaagaagtctatgctacagaaactattacgctgacaaccagacctgcgatggagaactcctgttcaacatgaccaagaagatgtgctgttgctcctacaacatcggcagagcctggaacaaaccctgtgaacagtgccccatcccaagcacagatgagtttgctaccctctgtgggagccagaggcccggcttcgtgattgacatttatacgggtttacccgtggatattgatgaatgccgggagatccctggggtctgtgaaaatggagtgtgcatcaacatggttggcagcttccggtgtgagtgtcccgtgggattcttctataacgacaagttactggtttgtgaagatatcgacgagtgtcagaatggccctgtgtgccagcgaaatgcggaatgcatcaacactgcaggcagctaccgctgtgactgtaagcccggctaccgccttacctccacaggtcaatgcaacgatcgaaacgagtgccaagaaatcccgaacatatgcagtcatggccagtgcatcgacaccgtgggaagcttctactgcctttgtcacactggcttcaaaacaaatgtggatcagaccatgtgcttagacataaatgagtgtgagagagacgcctgtgggaacgggacttgcagaaacacgattggctccttcaactgtcgctgtaaccatggcttcatactgtctcacaacaatgactgcatagatgttgatgagtgtgcaactggaaacgggaacctttgcagaaatggccagtgtgtcaataccgtgggctcctttcagtgcaggtgcaatgaaggctatgaggtggctccggacggcaggacctgtgtggatatcaacgagtgtgttctggatcctgggaaatgtgcacctggaacctgtcagaacctggatggctcctacagatgcatttgcccgcctgggtatagtctacagaatgacaagtgtgaagatattgatgagtgtgttgaagagccagaaatctgtgccttggggacctgcagcaacactgagggtagcttcaaatgtctgtgtccagaggggttctccctgtcctccactggaagaaggtgccaagatttgcgaatgagctactgctatgcgaagtttgaaggtgggaagtgttcatcacccaaatccagaaaccattccaagcaggagtgctgctgtgctttgaagggagaaggctggggagatccttgtgagttgtgccccactgagccagatgaggctttccgccagatctgcccctttggaagtgggatcattgtgggccctgatgactcagcagttgatatggacgaatgcaaagaacctgatgtctgtagacatgggcagtgcattaacacagacggctcctatcgatgcgagtgtccttttggttatattctggaagggaatgagtgtgtggataccgatgaatgctctgtgggcaatccttgtggaaatgggacctgcaagaatgtgattggaggttttgaatgtacctgtgaggaggggttcgagcctggcccaatgatgacttgtgaagatataaatgaatgtgcccagaatcctctgctctgcgccttccgctgtgtaaatacctacgggtcctatgaatgcaaatgccctgttggatacgttctccgagaagacaggaggatgtgtaaagatgaggatgagtgtgcagagggaaaacacgactgtactgagaagcaaatggagtgtaagaacctcattggtacctacatgtgcatctgcggccctgggtaccagcgcagacccgatggagagggctgcatagatgagaatgagtgtcagaccaagcccgggatctgtgagaatgggcgttgcctcaacaccctgggtagctacacttgtgagtgtaacgatggcttcacagccagccccactcaggatgagtgcttggacaaccgggaagggtactgcttttcggaggtcttgcaaaacatgtgccagattggctcaagcaacaggaaccccgtcaccaagtccgagtgctgctgtgatggagggagaggctggggaccccactgtgagatctgccctttcgagggcacagtggcttacaagaagctctgtccccacggccgaggattcatgaccaacggagcagatattgatgagtgcaaggttattcatgatgtttgccgaaatggggagtgtgtcaacgacagagggtcctatcactgcatctgtaaaactggctacactccggatataacagggaccgcctgtgtagatctgaatgaatgcaaccaggctcccaaaccctgcaattttatatgcaaaaacacagaagggagttaccagtgttcctgcccgaagggctacattctgcaagaggatggaaggagctgcaaagatcttgacgagtgtgcaaccaagcagcataactgtcagttcctgtgtgttaacaccatcggtggcttcacatgcaaatgccctcctgggtttacccagcatcacactgcctgcattgataacaatgagtgcacgtctgatatcaacctgtgtgggtccaagggtgtttgccagaacactccaggaagcttcacctgtgaatgccaacgggggttctcactcgatcagagtggtgccagctgtgaagatgtggacgagtgtgagggtaaccaccgctgtcaacatggctgccagaacatcatcggaggctataggtgtagctgcccccagggctacctccagcactaccaatggaaccagtgtgtagatgaaaacgagtgcctgagtgcacatgtctgtggaggagcctcctgccacaacaccctggggagttacaagtgcatgtgtcccaccggcttccagtacgaacagttcagtggaggctgccaagacatcaatgagtgtggctcatcccaggccccctgcagttacggttgctctaatactgagggtggctacctgtgtggctgtccaccaggatacttccggataggccaagggcattgtgtttctggaatgggcatgggccgaggcggcccagagccacctgccagcagcgagatggacgacaactcactgtccccagaggcctgctatgagtgtgatcaatggctaccccaaacggggcaggaaacggagaagcacaaacgaaactgatgcctccgacatccaggacgggtctgagatggaagccaacgtgagcctcgccagctgggatgtggagaagccggctagctttgctttcaatatttcccatgtcaataacaaggtccgaatcctagagctcctgccggccctcacaactctgatgaaccacaacagatacttgattgaatctggaaatgaagatggcttctttaaaatcaaccagaaagaaggggtcagctacctccacttcacgaagaagaagccggtggctgggacctactccttacaaatcagcagcaccccactttataaaaagaaagaacttaaccagttagaagacagatatgacaaagactacctcagtggtgaactgggcgataacctgaagatgaaaattcagatcttgctgcattaa

SEQ ID NO: 24 - DNA, 175 bp, Homo sapiens
gcactgtgtttctggaatgggcatgggccgaggaaacccagagccacctgtcagtggtgaaatggatgacaattcactctccccagaggcttgttacgagtgtaagatcaatggctaccccaaacggggcaggaaacggagaagcacaaacgaaactgatgcctccaatatcgag

SEQ ID NO: 25 - DNA, 175 bp, Mus musculus
gcattgtgtttctggaatgggcatgggccgaggcggcccagagccacctgccagcagcgagatggacgacaactcactgtccccagaggcctgctatgagtgtaagatcaacggctacccaaaacgaggccggaaacggagaagcacgaacgaaacggatgcctccgacatccag

SEQ ID NO: 26 - DNA, 176 bp, Artificial Sequence
  Synthetic
gcattgtgtttctggaatgggcatgggccgaggcggcccagagccacctgccagcagcgagatggacgacaactcactgtccccagaggcctgctatgagtgtaagatcaacggctacccaaaacgaggccggaaacggagaagcacgaacgaaaactgatgcctccgacatccag

SEQ ID NO: 27 - DNA, 200 bp, Artificial Sequence
  Synthetic
gcattgtgtttctggaatgggcatgggccgaggcggcccagagccacctgccagcagcgagatggacgacaactcactgtccccagaggcctgctatgagtgtaagatcaacggctacccaaaggcggcccagagccacctgccagcaacgaggccggaaacggagaagcacgaacgaaacggatgcctccgacatccag

SEQ ID NO: 28 - DNA, 173 bp, Artificial Sequence
  Synthetic
gcattgtgtttctggaatgggcatgggccgaggcggcccagagccacctgccagcagcgagatggacgacaactcactgtccccagaggcctgctatgagtgtgatcaatggctaccccaaacggggcaggaaacggagaagcacaaacgaaactgatgcctccgacatccag

SEQ ID NO: 29 - protein, 2871 aa, Homo sapiens
MRRGRLLEIALGFTVLLASYTSHGADANLEAGNVKETRASRAKRRGGGGHDALKGPNVCGSRYNAYCCPGWKTLPGGNQCIVPICRHSCGDGFCSRPNMCTCPSGQIAPSCGSRSIQHCNIRCMNGGSCSDDHCLCQKGYIGTHCGQPVCESGCLNGGRCVAPNRCACTYGFTGPQCERDYRTGPCFTVISNQMCQGQLSGIVCTKTLCCATVGRAWGHPCEMCPAQPHPCRRGFIPNIRTGACQDVDECQAIPGLCQGGNCINTVGSFECKCPAGHKLNEVSQKCEDIDECSTIPGICEGGECTNTVSSYFCKCPPGFYTSPDGTRCIDVRPGYCYTALTNGRCSNQLPQSITKMQCCCDAGRCWSPGVTVAPEMCPIRATEDFNKLCSVPMVIPGRPEYPPPPLGPIPPVLPVPPGFPPGPQIPVPRPPVEYLYPSREPPRVLPVNVTDYCQLVRYLCQNGRCIPTPGSYRCECNKGFQLDLRGECIDVDECEKNPCAGGECINNQGSYTCQCRAGYQSTLTRTECRDIDECLQNGRICNNGRCINTDGSFHCVCNAGFHVTRDGKNCEDMDECSIRNMCLNGMCINEDGSFKCICKPGFQLASDGRYCKDINECETPGICMNGRCVNTDGSYRCECFPGLAVGLDGRVCVDTHMRSTCYGGYKRGQCIKPLFGAVTKSECCCASTEYAFGEPCQPCPAQNSAEYQALCSSGPGMTSAGSDINECALDPDICPNGICENLRGTYKCICNSGYEVDSTGKNCVDINECVLNSLLCDNGQCRNTPGSFVCTCPKGFIYKPDLKTCEDIDECESSPCINGVCKNSPGSFICECSSESTLDPTKTICIETIKGTCWQTVIDGRCEININGATLKSQCCSSLGAAWGSPCTLCQVDPICGKGYSRIKGTQCEDIDECEVFPGVCKNGLCVNTRGSFKCQCPSGMTLDATGRICLDIRLETCFLRYEDEECTLPIAGRHRMDACCCSVGAAWGTEECEECPMRNTPEYEELCPRGPGFATKEITNGKPFFKDINECKMIPSLCTHGKCRNTIGSFKCRCDSGFALDSEERNCTDIDECRISPDLCGRGQCVNTPGDFECKCDEGYESGFMMMKNCMDIDECQRDPLLCRGGVCHNTEGSYRCECPPGHQLSPNISACIDINECELSAHLCPNGRCVNLIGKYQCACNPGYHSTPDRLFCVDIDECSIMNGGCETFCTNSEGSYECSCQPGFALMPDQRSCTDIDECEDNPNICDGGQCTNIPGEYRCLCYDGFMASEDMKTCVDVNECDLNPNICLSGTCENTKGSFICHCDMGYSGKKGKTGCTDINECEIGAHNCGKHAVCTNTAGSFKCSCSPGWIGDGIKCTDLDECSNGTHMCSQHADCKNTMGSYRCLCKEGYTGDGFTCTDLDECSENLNLCGNGQCLNAPGGYRCECDMGFVPSADGKACEDIDECSLPNICVFGTCHNLPGLFRCECEIGYELDRSGGNCTDVNECLDPTTCISGNCVNTPGSYICDCPPDFELNPTRVGCVDTRSGNCYLDIRPRGDNGDTACSNEIGVGVSKASCCCSLGKAWGTPCEMCPAVNTSEYKILCPGGEGFRPNPITVILEDIDECQELPGLCQGGKCINTFGSFQCRCPTGYYLNEDTRVCDDVNECETPGICGPGTCYNTVGNYTCICPPDYMQVNGGNNCMDMRRSLCYRNYYADNQTCDGELLFNMTKKMCCCSYNIGRAWNKPCEQCPIPSTDEFATLCGSQRPGFVIDIYTGLPVDIDECREIPGVCENGVCINMVGSFRCECPVGFFYNDKLLVCEDIDECQNGPVCQRNAECINTAGSYRCDCKPGYRFTSTGQCNDRNECQEIPNICSHGQCIDTVGSFYCLCHTGFKTNDDQTMCLDINECERDACGNGTCRNTIGSFNCRCNHGFILSHNNDCIDVDECASGNGNLCRNGQCINTVGSFQCQCNEGYEVAPDGRTCVDINECLLEPRKCAPGTCQNLDGSYRCICPPGYSLQNEKCEDIDECVEEPEICALGTCSNTEGSFKCLCPEGFSLSSSGRRCQDLRMSYCYAKFEGGKCSSPKSRNHSKQECCCALKGEGWGDPCELCPTEPDEAFRQICPYGSGIIVGPDDSAVDMDECKEPDVCKHGQCINTDGSYRCECPFGYILAGNECVDTDECSVGNPCGNGTCKNVIGGFECTCEEGFEPGPMMTCEDINECAQNPLLCAFRCVNTYGSYECKCPVGYVLREDRRMCKDEDECEEGKHDCTEKQMECKNLIGTYMCICGPGYQRRPDGEGCVDENECQTKPGICENGRCLNTRGSYTCECNDGFTASPNQDECLDNREGYCFTEVLQNMCQIGSSNRNPVTKSECCCDGGRGWGPHCEICPFQGTVAFKKLCPHGRGFMTNGADIDECKVIHDVCRNGECVNDRGSYHCICKTGYTPDITGTSCVDLNECNQAPKPCNFICKNTEGSYQCSCPKGYILQEDGRSCKDLDECATKQHNCQFLCVNTIGGFTCKCPPGFTQHHTSCIDNNECTSDINLCGSKGICQNTPGSFTCECQRGFSLDQTGSSCEDVDECEGNHRCQHGCQNIIGGYRCSCPQGYLQHYQWNQCVDENECLSAHICGGASCHNTLGSYKCMCPAGFQYEQFSGGCQDINECGSAQAPCSYGCSNTEGGYLCGCPPGYFRIGQGHCVSGMGMGRGNPEPPVSGEMDDNSLSPEACYECKINGYPKRGRKRRSTNETDASNIEDQSETEANVSLASWDVEKTAIFAFNISHVSNKVRILELLPALTTLTNHNRYLIESGNEDGFFKINQKEGISYLHFTKKKPVAGTYSLQISSTPLYKKKELNQLEDKYDKDYLSGELGDNLKMKIQVLLH

SEQ ID NO: 30 - protein, 2873 aa, Mus musculus
MRRGGLLEVALAFALLLESYTSHGADANLEAGSLKETRANRAKRRGGGGHDALKGPNVCGSRYNAYCCPGWKTLPGGNQCIVPICRHSCGDGFCSRPNMCTCPSGQISPSCGSRSIQHCSIRCMNGGSCSDDHCLCQKGYIGTHCGQPVCESGCLNGGRCVAPNRCACTYGFTGPQCERDYRTGPCFTVVSNQMCQGQLSGIVCTKTLCCATVGRAWGHPCEMCPAQPHPCRRGFIPNIRTGACQDVDECQAIPGMCQGGNCINTVGSFECKCPAGHKFNEVSQKCEDIDECSTIPGVCDGGECTNTVSSYFCKCPPGFYTSPDGTRCVDVRPGYCYTALANGRCSNQLPQSITKMQCCCDLGRCWSPGVTVAPEMCPIRSTEDFNKLCSVPLVIPGRPEYPPPPIGPLPPVQPVPPGYPPGPVIPAPRPPPEYPYPSPSREPPRVLPFNVTDYCQLVRYLCQNGRCIPTPGSYRCECNKGFQLDIRGECIDVDECEKNPCTGGECINNQGSYTCHCRAGYQSTLTRTECRDIDECLQNGRICNNGRCINTDGSFHCVCNAGFHVTRDGKNCEDMDECSIRNMCLNGMCINEDGSFKCICKPGFQLASDGRYCKDINECETPGICMNGRCVNTDGSYRCECFPGLAVGLDGRVCVDTHMRSTCYGGYRRGQCVKPLFGAVTKSECCCASTEYAFGEPCQPCPAQNSAEYQALCSSGPGMTSAGTDINECALDPDICPNGICENLRGTYKCICNSGYEVDITGKNCVDINECVLNSLLCDNGQCRNTPGSFVCTCPKGFVYKPDLKTCEDIDECESSPCINGVCKNSPGSFICECSPESTLDPTKTICIETIKGTCWQTVIDGRCEININGATLKSECCSSLGAAWGSPCTICQLDPICGKGFSRIKGTQCEDINECEVFPGVCKNGLCVNSRGSFKCECPNGMTLDATGRICLDIRLETCFLKYDDEECTLPIAGRHRMDACCCSVGAAWGTEECEECPLRNSREYEELCPRGPGFATKDITNGKPFFKDINECKMIPSLCTHGKCRNTIGSFKCRCDSGFALDSEERNCTDIDECRISPDLCGRGQCVNTPGDFECKCDEGYESGFMMMKNCMDIDECQRDPLLCRGGICHNTEGSYRCECPPGHQLSPNISACIDINECELSANLCPHGRCVNLIGKYQCACNPGYHPTHDRLFCVDIDECSIMNGGCETFCTNSDGSYECSCQPGFALMPDQRSCTDIDECEDNPNICDGGQCTNIPGEYRCLCYDGFMASEDMKTCVDVNECDLNPNICLSGTCENTKGSFICHCDMGYSGKKGKTGCTDINECEIGAHNCGRHAVCTNTAGSFKCSCSPGWIGDGIKCTDLDECSNGTHMCSQHADCKNTMGSYRCLCKDGYTGDGFTCTDLDECSENLNLCGNGQCLNAPGGYRCECDMGFVPSADGKACEDIDECSLPNICVFGTCHNLPGLFRCECEIGYELDRSGGNCTDVNECLDPTTCISGNCVNTPGSYTCDCPPDFELNPTRVGCVDTRSGNCYLDIRPRGDNGDTACSNEIGVGVSKASCCCSLGKAWGTPCELCPSVNTSEYKILCPGGEGFRPNPITVILEDIDECQELPGLCQGGKCINTFGSFQCRCPTGYYLNEDTRVCDDVNECETPGICGPGTCYNTVGNYTCICPPDYMQVNGGNNCMDMRRSLCYRNYYADNQTCDGELLFNMTKKMCCCSYNIGRAWNKPCEQCPIPSTDEFATLCGSQRPGFVIDIYTGLPVDIDECREIPGVCENGVCINMVGSFRCECPVGFFYNDKLLVCEDIDECQNGPVCQRNAECINTAGSYRCDCKPGYRLTSTGQCNDRNECQEIPNICSHGQCIDTVGSFYCLCHTGFKTNVDQTMCLDINECERDACGNGTCRNTIGSFNCRCNHGFILSHNNDCIDVDECATGNGNLCRNGQCVNTVGSFQCRCNEGYEVAPDGRTCVDINECVLDPGKCAPGTCQNLDGSYRCICPPGYSLQNDKCEDIDECVEEPEICALGTCSNTEGSFKCLCPEGFSLSSTGRRCQDLRMSYCYAKFEGGKCSSPKSRNHSKQECCCALKGEGWGDPCELCPTEPDEAFRQICPFGSGIIVGPDDSAVDMDECKEPDVCRHGQCINTDGSYRCECPFGYILEGNECVDTDECSVGNPCGNGTCKNVIGGFECTCEEGFEPGPMMTCEDINECAQNPLLCAFRCVNTYGSYECKCPVGYVLREDRRMCKDEDECAEGKHDCTEKQMECKNLIGTYMCICGPGYQRRPDGEGCIDENECQTKPGICENGRCLNTLGSYTCECNDGFTASPTQDECLDNREGYCFSEVLQNMCQIGSSNRNPVTKSECCCDGGRGWGPHCEICPFEGTVAYKKLCPHGRGFMTNGADIDECKVIHDVCRNGECVNDRGSYHCICKTGYTPDITGTACVDLNECNQAPKPCNFICKNTEGSYQCSCPKGYILQEDGRSCKDLDECATKQHNCQFLCVNTIGGFTCKCPPGFTQHHTACIDNNECTSDINLCGSKGVCQNTPGSFTCECQRGFSLDQSGASCEDVDECEGNHRCQHGCQNIIGGYRCSCPQGYLQHYQWNQCVDENECLSAHVCGGASCHNTLGSYKCMCPTGFQYEQFSGGCQDINECGSSQAPCSYGCSNTEGGYLCGCPPGYFRIGQGHCVSGMGMGRGGPEPPASSEMDDNSLSPEACYECKINGYPKRGRKRRSTNETDASDIQDGSEMEANVSLASWDVEKPASFAFNISHVNNKVRILELLPALTTLMNHNRYLIESGNEDGFFKINQKEGVSYLHFTKKKPVAGTYSLQISSTPLYKKKELNQLEDRYDKDYLSGELGDNLKMKIQILLH

SEQ ID NO: 31 - protein, 2738 aa, Artificial Sequence
  Synthetic
MRRGGLLEVALAFALLLESYTSHGADANLEAGSLKETRANRAKRRGGGGHDALKGPNVCGSRYNAYCCPGWKTLPGGNQCIVPICRHSCGDGFCSRPNMCTCPSGQISPSCGSRSIQHCSIRCMNGGSCSDDHCLCQKGYIGTHCGQPVCESGCLNGGRCVAPNRCACTYGFTGPQCERDYRTGPCFTVVSNQMCQGQLSGIVCTKTLCCATVGRAWGHPCEMCPAQPHPCRRGFIPNIRTGACQDVDECQAIPGMCQGGNCINTVGSFECKCPAGHKFNEVSQKCEDIDECSTIPGVCDGGECTNTVSSYFCKCPPGFYTSPDGTRCVDVRPGYCYTALANGRCSNQLPQSITKMQCCCDLGRCWSPGVTVAPEMCPIRSTEDFNKLCSVPLVIPGRPEYPPPPIGPLPPVQPVPPGYPPGPVIPAPRPPPEYPYPSPSREPPRVLPFNVTDYCQLVRYLCQNGRCIPTPGSYRCECNKGFQLDIRGECIDVDECEKNPCTGGECINNQGSYTCHCRAGYQSTLTRTECRDIDECLQNGRICNNGRCINTDGSFHCVCNAGFHVTRDGKNCEDMDECSIRNMCLNGMCINEDGSFKCICKPGFQLASDGRYCKDINECETPGICMNGRCVNTDGSYRCECFPGLAVGLDGRVCVDTHMRSTCYGGYRRGQCVKPLFGAVTKSECCCASTEYAFGEPCQPCPAQNSAEYQALCSSGPGMTSAGTDINECALDPDICPNGICENLRGTYKCICNSGYEVDITGKNCVDINECVLNSLLCDNGQCRNTPGSFVCTCPKGFVYKPDLKTCEDIDECESSPCINGVCKNSPGSFICECSPESTLDPTKTICIETIKGTCWQTVIDGRCEININGATLKSECCSSLGAAWGSPCTICQLDPICGKGFSRIKGTQCEDINECEVFPGVCKNGLCVNSRGSFKCECPNGMTLDATGRICLDIRLETCFLKYDDEECTLPIAGRHRMDACCCSVGAAWGTEECEECPLRNSREYEELCPRGPGFATKDITNGKPFFKDINECKMIPSLCTHGKCRNTIGSFKCRCDSGFALDSEERNCTDIDECRISPDLCGRGQCVNTPGDFECKCDEGYESGFMMMKNCMDIDECQRDPLLCRGGICHNTEGSYRCECPPGHQLSPNISACIDINECELSANLCPHGRCVNLIGKYQCACNPGYHPTHDRLFCVDIDECSIMNGGCETFCTNSDGSYECSCQPGFALMPDQRSCTDIDECEDNPNICDGGQCTNIPGEYRCLCYDGFMASEDMKTCVDVNECDLNPNICLSGTCENTKGSFICHCDMGYSGKKGKTGCTDINECEIGAHNCGRHAVCTNTAGSFKCSCSPGWIGDGIKCTDLDECSNGTHMCSQHADCKNTMGSYRCLCKDGYTGDGFTCTDLDECSENLNLCGNGQCLNAPGGYRCECDMGFVPSADGKACEDIDECSLPNICVFGTCHNLPGLFRCECEIGYELDRSGGNCTDVNECLDPTTCISGNCVNTPGSYTCDCPPDFELNPTRVGCVDTRSGNCYLDIRPRGDNGDTACSNEIGVGVSKASCCCSLGKAWGTPCELCPSVNTSEYKILCPGGEGFRPNPITVILEDIDECQELPGLCQGGKCINTFGSFQCRCPTGYYLNEDTRVCDDVNECETPGICGPGTCYNTVGNYTCICPPDYMQVNGGNNCMDMRRSLCYRNYYADNQTCDGELLFNMTKKMCCCSYNIGRAWNKPCEQCPIPSTDEFATLCGSQRPGFVIDIYTGLPVDIDECREIPGVCENGVCINMVGSFRCECPVGFFYNDKLLVCEDIDECQNGPVCQRNAECINTAGSYRCDCKPGYRLTSTGQCNDRNECQEIPNICSHGQCIDTVGSFYCLCHTGFKTNVDQTMCLDINECERDACGNGTCRNTIGSFNCRCNHGFILSHNNDCIDVDECATGNGNLCRNGQCVNTVGSFQCRCNEGYEVAPDGRTCVDINECVLDPGKCAPGTCQNLDGSYRCICPPGYSLQNDKCEDIDECVEEPEICALGTCSNTEGSFKCLCPEGFSLSSTGRRCQDLRMSYCYAKFEGGKCSSPKSRNHSKQECCCALKGEGWGDPCELCPTEPDEAFRQICPFGSGIIVGPDDSAVDMDECKEPDVCRHGQCINTDGSYRCECPFGYILEGNECVDTDECSVGNPCGNGTCKNVIGGFECTCEEGFEPGPMMTCEDINECAQNPLLCAFRCVNTYGSYECKCPVGYVLREDRRMCKDEDECAEGKHDCTEKQMECKNLIGTYMCICGPGYQRRPDGEGCIDENECQTKPGICENGRCLNTLGSYTCECNDGFTASPTQDECLDNREGYCFSEVLQNMCQIGSSNRNPVTKSECCCDGGRGWGPHCEICPFEGTVAYKKLCPHGRGFMTNGADIDECKVIHDVCRNGECVNDRGSYHCICKTGYTPDITGTACVDLNECNQAPKPCNFICKNTEGSYQCSCPKGYILQEDGRSCKDLDECATKQHNCQFLCVNTIGGFTCKCPPGFTQHHTACIDNNECTSDINLCGSKGVCQNTPGSFTCECQRGFSLDQSGASCEDVDECEGNHRCQHGCQNIIGGYRCSCPQGYLQHYQWNQCVDENECLSAHVCGGASCHNTLGSYKCMCPTGFQYEQFSGGCQDINECGSSQAPCSYGCSNTEGGYLCGCPPGYFRIGQGHCVSGMGMGRGGPEPPASSEMDDNSLSPEACYECKINGYPKRGRKRRSTNEN

SEQ ID NO: 32 - protein, 2755 aa, Artificial Sequence
  Synthetic
MRRGGLLEVALAFALLLESYTSHGADANLEAGSLKETRANRAKRRGGGGHDALKGPNVCGSRYNAYCCPGWKTLPGGNQCIVPICRHSCGDGFCSRPNMCTCPSGQISPSCGSRSIQHCSIRCMNGGSCSDDHCLCQKGYIGTHCGQPVCESGCLNGGRCVAPNRCACTYGFTGPQCERDYRTGPCFTVVSNQMCQGQLSGIVCTKTLCCATVGRAWGHPCEMCPAQPHPCRRGFIPNIRTGACQDVDECQAIPGMCQGGNCINTVGSFECKCPAGHKFNEVSQKCEDIDECSTIPGVCDGGECTNTVSSYFCKCPPGFYTSPDGTRCVDVRPGYCYTALANGRCSNQLPQSITKMQCCCDLGRCWSPGVTVAPEMCPIRSTEDFNKLCSVPLVIPGRPEYPPPPIGPLPPVQPVPPGYPPGPVIPAPRPPPEYPYPSPSREPPRVLPFNVTDYCQLVRYLCQNGRCIPTPGSYRCECNKGFQLDIRGECIDVDECEKNPCTGGECINNQGSYTCHCRAGYQSTLTRTECRDIDECLQNGRICNNGRCINTDGSFHCVCNAGFHVTRDGKNCEDMDECSIRNMCLNGMCINEDGSFKCICKPGFQLASDGRYCKDINECETPGICMNGRCVNTDGSYRCECFPGLAVGLDGRVCVDTHMRSTCYGGYRRGQCVKPLFGAVTKSECCCASTEYAFGEPCQPCPAQNSAEYQALCSSGPGMTSAGTDINECALDPDICPNGICENLRGTYKCICNSGYEVDITGKNCVDINECVLNSLLCDNGQCRNTPGSFVCTCPKGFVYKPDLKTCEDIDECESSPCINGVCKNSPGSFICECSPESTLDPTKTICIETIKGTCWQTVIDGRCEININGATLKSECCSSLGAAWGSPCTICQLDPICGKGFSRIKGTQCEDINECEVFPGVCKNGLCVNSRGSFKCECPNGMTLDATGRICLDIRLETCFLKYDDEECTLPIAGRHRMDACCCSVGAAWGTEECEECPLRNSREYEELCPRGPGFATKDITNGKPFFKDINECKMIPSLCTHGKCRNTIGSFKCRCDSGFALDSEERNCTDIDECRISPDLCGRGQCVNTPGDFECKCDEGYESGFMMMKNCMDIDECQRDPLLCRGGICHNTEGSYRCECPPGHQLSPNISACIDINECELSANLCPHGRCVNLIGKYQCACNPGYHPTHDRLFCVDIDECSIMNGGCETFCTNSDGSYECSCQPGFALMPDQRSCTDIDECEDNPNICDGGQCTNIPGEYRCLCYDGFMASEDMKTCVDVNECDLNPNICLSGTCENTKGSFICHCDMGYSGKKGKTGCTDINECEIGAHNCGRHAVCTNTAGSFKCSCSPGWIGDGIKCTDLDECSNGTHMCSQHADCKNTMGSYRCLCKDGYTGDGFTCTDLDECSENLNLCGNGQCLNAPGGYRCECDMGFVPSADGKACEDIDECSLPNICVFGTCHNLPGLFRCECEIGYELDRSGGNCTDVNECLDPTTCISGNCVNTPGSYTCDCPPDFELNPTRVGCVDTRSGNCYLDIRPRGDNGDTACSNEIGVGVSKASCCCSLGKAWGTPCELCPSVNTSEYKILCPGGEGFRPNPITVILEDIDECQELPGLCQGGKCINTFGSFQCRCPTGYYLNEDTRVCDDVNECETPGICGPGTCYNTVGNYTCICPPDYMQVNGGNNCMDMRRSLCYRNYYADNQTCDGELLFNMTKKMCCCSYNIGRAWNKPCEQCPIPSTDEFATLCGSQRPGFVIDIYTGLPVDIDECREIPGVCENGVCINMVGSFRCECPVGFFYNDKLLVCEDIDECQNGPVCQRNAECINTAGSYRCDCKPGYRLTSTGQCNDRNECQEIPNICSHGQCIDTVGSFYCLCHTGFKTNVDQTMCLDINECERDACGNGTCRNTIGSFNCRCNHGFILSHNNDCIDVDECATGNGNLCRNGQCVNTVGSFQCRCNEGYEVAPDGRTCVDINECVLDPGKCAPGTCQNLDGSYRCICPPGYSLQNDKCEDIDECVEEPEICALGTCSNTEGSFKCLCPEGFSLSSTGRRCQDLRMSYCYAKFEGGKCSSPKSRNHSKQECCCALKGEGWGDPCELCPTEPDEAFRQICPFGSGIIVGPDDSAVDMDECKEPDVCRHGQCINTDGSYRCECPFGYILEGNECVDTDECSVGNPCGNGTCKNVIGGFECTCEEGFEPGPMMTCEDINECAQNPLLCAFRCVNTYGSYECKCPVGYVLREDRRMCKDEDECAEGKHDCTEKQMECKNLIGTYMCICGPGYQRRPDGEGCIDENECQTKPGICENGRCLNTLGSYTCECNDGFTASPTQDECLDNREGYCFSEVLQNMCQIGSSNRNPVTKSECCCDGGRGWGPHCEICPFEGTVAYKKLCPHGRGFMTNGADIDECKVIHDVCRNGECVNDRGSYHCICKTGYTPDITGTACVDLNECNQAPKPCNFICKNTEGSYQCSCPKGYILQEDGRSCKDLDECATKQHNCQFLCVNTIGGFTCKCPPGFTQHHTACIDNNECTSDINLCGSKGVCQNTPGSFTCECQRGFSLDQSGASCEDVDECEGNHRCQHGCQNIIGGYRCSCPQGYLQHYQWNQCVDENECLSAHVCGGASCHNTLGSYKCMCPTGFQYEQFSGGCQDINECGSSQAPCSYGCSNTEGGYLCGCPPGYFRIGQGHCVSGMGMGRGGPEPPASSEMDDNSLSPEACYECKINGYPKAAQSHLPATRPETEKHERNGCLRHPGRV

SEQ ID NO: 33 - protein, 2737 aa, Artificial Sequence
  Synthetic
MRRGGLLEVALAFALLLESYTSHGADANLEAGSLKETRANRAKRRGGGGHDALKGPNVCGSRYNAYCCPGWKTLPGGNQCIVPICRHSCGDGFCSRPNMCTCPSGQISPSCGSRSIQHCSIRCMNGGSCSDDHCLCQKGYIGTHCGQPVCESGCLNGGRCVAPNRCACTYGFTGPQCERDYRTGPCFTVVSNQMCQGQLSGIVCTKTLCCATVGRAWGHPCEMCPAQPHPCRRGFIPNIRTGACQDVDECQAIPGMCQGGNCINTVGSFECKCPAGHKFNEVSQKCEDIDECSTIPGVCDGGECTNTVSSYFCKCPPGFYTSPDGTRCVDVRPGYCYTALANGRCSNQLPQSITKMQCCCDLGRCWSPGVTVAPEMCPIRSTEDFNKLCSVPLVIPGRPEYPPPPIGPLPPVQPVPPGYPPGPVIPAPRPPPEYPYPSPSREPPRVLPFNVTDYCQLVRYLCQNGRCIPTPGSYRCECNKGFQLDIRGECIDVDECEKNPCTGGECINNQGSYTCHCRAGYQSTLTRTECRDIDECLQNGRICNNGRCINTDGSFHCVCNAGFHVTRDGKNCEDMDECSIRNMCLNGMCINEDGSFKCICKPGFQLASDGRYCKDINECETPGICMNGRCVNTDGSYRCECFPGLAVGLDGRVCVDTHMRSTCYGGYRRGQCVKPLFGAVTKSECCCASTEYAFGEPCQPCPAQNSAEYQALCSSGPGMTSAGTDINECALDPDICPNGICENLRGTYKCICNSGYEVDITGKNCVDINECVLNSLLCDNGQCRNTPGSFVCTCPKGFVYKPDLKTCEDIDECESSPCINGVCKNSPGSFICECSPESTLDPTKTICIETIKGTCWQTVIDGRCEININGATLKSECCSSLGAAWGSPCTICQLDPICGKGFSRIKGTQCEDINECEVFPGVCKNGLCVNSRGSFKCECPNGMTLDATGRICLDIRLETCFLKYDDEECTLPIAGRHRMDACCCSVGAAWGTEECEECPLRNSREYEELCPRGPGFATKDITNGKPFFKDINECKMIPSLCTHGKCRNTIGSFKCRCDSGFALDSEERNCTDIDECRISPDLCGRGQCVNTPGDFECKCDEGYESGFMMMKNCMDIDECQRDPLLCRGGICHNTEGSYRCECPPGHQLSPNISACIDINECELSANLCPHGRCVNLIGKYQCACNPGYHPTHDRLFCVDIDECSIMNGGCETFCTNSDGSYECSCQPGFALMPDQRSCTDIDECEDNPNICDGGQCTNIPGEYRCLCYDGFMASEDMKTCVDVNECDLNPNICLSGTCENTKGSFICHCDMGYSGKKGKTGCTDINECEIGAHNCGRHAVCTNTAGSFKCSCSPGWIGDGIKCTDLDECSNGTHMCSQHADCKNTMGSYRCLCKDGYTGDGFTCTDLDECSENLNLCGNGQCLNAPGGYRCECDMGFVPSADGKACEDIDECSLPNICVFGTCHNLPGLFRCECEIGYELDRSGGNCTDVNECLDPTTCISGNCVNTPGSYTCDCPPDFELNPTRVGCVDTRSGNCYLDIRPRGDNGDTACSNEIGVGVSKASCCCSLGKAWGTPCELCPSVNTSEYKILCPGGEGFRPNPITVILEDIDECQELPGLCQGGKCINTFGSFQCRCPTGYYLNEDTRVCDDVNECETPGICGPGTCYNTVGNYTCICPPDYMQVNGGNNCMDMRRSLCYRNYYADNQTCDGELLFNMTKKMCCCSYNIGRAWNKPCEQCPIPSTDEFATLCGSQRPGFVIDIYTGLPVDIDECREIPGVCENGVCINMVGSFRCECPVGFFYNDKLLVCEDIDECQNGPVCQRNAECINTAGSYRCDCKPGYRLTSTGQCNDRNECQEIPNICSHGQCIDTVGSFYCLCHTGFKTNVDQTMCLDINECERDACGNGTCRNTIGSFNCRCNHGFILSHNNDCIDVDECATGNGNLCRNGQCVNTVGSFQCRCNEGYEVAPDGRTCVDINECVLDPGKCAPGTCQNLDGSYRCICPPGYSLQNDKCEDIDECVEEPEICALGTCSNTEGSFKCLCPEGFSLSSTGRRCQDLRMSYCYAKFEGGKCSSPKSRNHSKQECCCALKGEGWGDPCELCPTEPDEAFRQICPFGSGIIVGPDDSAVDMDECKEPDVCRHGQCINTDGSYRCECPFGYILEGNECVDTDECSVGNPCGNGTCKNVIGGFECTCEEGFEPGPMMTCEDINECAQNPLLCAFRCVNTYGSYECKCPVGYVLREDRRMCKDEDECAEGKHDCTEKQMECKNLIGTYMCICGPGYQRRPDGEGCIDENECQTKPGICENGRCLNTLGSYTCECNDGFTASPTQDECLDNREGYCFSEVLQNMCQIGSSNRNPVTKSECCCDGGRGWGPHCEICPFEGTVAYKKLCPHGRGFMTNGADIDECKVIHDVCRNGECVNDRGSYHCICKTGYTPDITGTACVDLNECNQAPKPCNFICKNTEGSYQCSCPKGYILQEDGRSCKDLDECATKQHNCQFLCVNTIGGFTCKCPPGFTQHHTACIDNNECTSDINLCGSKGVCQNTPGSFTCECQRGFSLDQSGASCEDVDECEGNHRCQHGCQNIIGGYRCSCPQGYLQHYQWNQCVDENECLSAHVCGGASCHNTLGSYKCMCPTGFQYEQFSGGCQDINECGSSQAPCSYGCSNTEGGYLCGCPPGYFRIGQGHCVSGMGMGRGGPEPPASSEMDDNSLSPEACYECDQWLPQTGQETEKHKRN

SEQ ID NO: 34 - protein, 8 aa, Artificial Sequence
  Synthetic
ETEKHKRN

SEQ ID NO: 35 - protein, 8 aa, Artificial Sequence
  Synthetic
ISLRQKPM

SEQ ID NO: 36 - protein, 6 aa, Artificial Sequence
  Synthetic
RGRKRR

SEQ ID NO: 37 - RNA, 23 nt, Artificial Sequence
  Synthetic
acggagaagcacgaacgaaacgg

SEQ ID NO: 38 - DNA, 123 bp, Artificial Sequence
  Synthetic
cagggcccttaggtatctgcagacaaggagaccctgatatacctggatgtcggaggcatcagttttcgttcgtgcttctccgtttccggcctcgttttgggtagccgttgatcttacactcat

SEQ ID NO: 39 - DNA, 23 bp, Artificial Sequence
  Synthetic
  misc_feature (2)..(21): n = A, T, C, or G
gnnnnnnnnnnnnnnnnnnnngg

SEQ ID NO: 40 - DNA, 23 bp, Artificial Sequence
  Synthetic
  misc_feature (1)..(21): n = A, T, C, or G
nnnnnnnnnnnnnnnnnnnnngg

SEQ ID NO: 41 - DNA, 25 bp, Artificial Sequence
  Synthetic
  misc_feature (3)..(23): n = A, T, C, or G
ggnnnnnnnnnnnnnnnnnnnnngg

SEQ ID NO: 42 - protein, 28 aa, Artificial Sequence
  Synthetic
AAQSHLPATRPETEKHERNGCLRHPGRV

SEQ ID NO: 43 - protein, 17 aa, Artificial Sequence
  Synthetic
DQWLPQTGQETEKHKRN

SEQ ID NO: 44 - DNA, 25 bp, Artificial Sequence
  Synthetic
aggcggcccagagccacctgccagc

SEQ ID NO: 45 - protein, 14 aa, Artificial Sequence
  Synthetic
YPKRGRKRRSTNEN

SEQ ID NO: 46 - protein, 14 aa, Artificial Sequence
  Synthetic
LPQTGQETEKHKRN

SEQ ID NO: 47 - protein, 14 aa, Artificial Sequence
  Synthetic
KHERNGCLRHPGRV